European Patent Application EP 4 524 163 A2, published March 19, 2025. Title: T CELL RECRUITING POLYPEPTIDES BASED ON TCR ALPHA/BETA REACTIVITY. Applicant: Ablynx N.V. The sequence listing filed with the application follows.

SEQUENCE LISTING (487 sequences)

SEQ ID NO: 1 - protein, 117 aa, synthetic construct
  REGION 1..117: note = Nanobody sequence
EVQLVESGGGLVQPGGSLRLSCAASGSVHKINFLGWYRQAPGKERELVATITIGDTTDYADSAKGRFTISRDEAKNMVYLQMNSLKPEDTAVHFCRAGSRLYPYNYWGQGTQVTVSS

SEQ ID NO: 2 - protein, 117 aa, synthetic construct
  REGION 1..117: note = Nanobody sequence
EVQLVESGGGLVQPGGSLRLSCAASGSVHKINFLGWYRQAPGKERGLVATITIGDTTDYADYAKGRFTISRDEARNMVYLQMNSLKPEDTAVYFCRAGSRLYPYNYWGQGTQVTVSS

SEQ ID NO: 3 - protein, 117 aa, synthetic construct
  REGION 1..117: note = Nanobody sequence
EVQLVESGGGLVQPGRSLRLPCAASGSVHKINFLGWYRQAPGKEREMVATITIGDATDYADSAKGRFTISRDEAKNMVYLQMNSLKPEDTAVYFCRAGSRLYPYNYWGQGTQVTVSS

SEQ ID NO: 4 - protein, 117 aa, synthetic construct
  REGION 1..117: note = Nanobody sequence
EVQLVESGGGLVQPGGSLRLSCAASGSVHKINFLGWYRQAPGKERELVATITIGDTTDYADYAKGRFTISRDEARNMVYLQMNSLKPEDTAVYFCRAGSRLYPYNYWGQGTLVTVSS

SEQ ID NO: 5 - protein, 117 aa, synthetic construct
  REGION 1..117: note = Nanobody sequence
EVQLVESGGGLVQPGGSLRLSCAASGSVHKINFLGWYRQAPGKEREMVATITIGDATDYADSAKGRFTISRDEAKNMVYLQMNSLKPEDTAVYFCRAGSRLYPYNYWGQGTLVTVSS

SEQ ID NO: 6 - protein, 117 aa, synthetic construct
  REGION 1..117: note = Nanobody sequence
EVQLVESGGGLVQPGGSLRLSCAASGSVHKINFLGWYRQAPGKERELVATITIGDTTDYADSAKGRFTISRDEAKNMVYLQMNSLKPEDTAVYFCRAGSRLYPYNYWGQGTQVTVSS

SEQ ID NO: 7 - protein, 117 aa, synthetic construct
  REGION 1..117: note = Nanobody sequence
EVQLVESGGGLVQPGGSLRLSCAVSGSVHLLNFLGWYRQAPGKEREMVAHITIADATDYSHFAKGRFTISRDEAKNMVYLQMNSLRPEDTAVYFCRAGSRIYPYDYWGQGTLVTVSS

SEQ ID NO: 8 - protein, 117 aa, synthetic construct
  REGION 1..117: note = Nanobody sequence
EVQLVESGGGLVQPGGSLKLSCAASGAVHKINFLGWYRQTPEKEREMVATITIGDDVDYADSAKGRFTISRDEAKNMVYLQMTSLKPEDTAVYVCRAGSRLYPYNYWGQGTLVTVSS

SEQ ID NO: 9 - protein, 117 aa, synthetic construct
  REGION 1..117: note = Nanobody sequence
EVQLVESGGGLVQPGGSLRLSCRASGDVHKINILGWYRQAPAKEREMVAHITIGDATDYAESAKGRFTISRDEAKNMVYLQMNSLKPEDTAVYFCRAYSRIYPYNYWGQGTQVTVSS

SEQ ID NO: 10 - protein, 117 aa, synthetic construct
  REGION 1..117: note = Nanobody sequence
EVQLVESGGGLVRPGGSLRLSCAASGDVHKINILGWYRQAPAKEREMVAHITIGDATDYADSAKGRFTISRDEAKNMVYLQMNSLKPEDTAVYFCRAYSRIYPYNYWGQGTLVTVSS

SEQ ID NO: 11 - protein, 117 aa, synthetic construct
  REGION 1..117: note = Nanobody sequence
EVQLVESGGGLVQPGGSLRLSCAASGDVHKINILGWYRQAPAKEREMVAHITIGDATDYADSAKGRFTISRDEAKNMVYLQMNSLKPEDTAVYFCRAYSRIYPYNYWGQGTLVTVSS

SEQ ID NO: 12 - protein, 117 aa, synthetic construct
  REGION 1..117: note = Nanobody sequence
EVQLVESGGGLVQPGGSLRLSCVASGDVHKINFLGWYRQAPGKEREKVAHITIGDQADYADSAKGRFTISRDEAKNMVYLQMNSLKPEDTAVYFCRAGSRIYPYDYWGQGTQVTVSS

SEQ ID NO: 13 - protein, 117 aa, synthetic construct
  REGION 1..117: note = Nanobody sequence
EVQLVESGGGSVQPGGSLRLSCAASGSVHKINFLGWYRQAPGKEREMVATITIGDATDYADSAKGRFTISRDEAKNMVYLQMNSLSPEDTAVYFCRAGSRLYPYNYWGQGTLVTVSS

SEQ ID NO: 14 - protein, 117 aa, synthetic construct
  REGION 1..117: note = Nanobody sequence
EVQLVESGGGLVQPGGSLRLSCAASGSVHLLNFLGWYRQAPGKEREMVAHISIADATDYAHFAKGRFTISRDEAKNMVYLQMNSLRPEDTAVYFCRAGSRIYPYDYWGRGTQVTVSS

SEQ ID NO: 15 - protein, 117 aa, synthetic construct
  REGION 1..117: note = Nanobody sequence
EVQLVESGGGLVQPGGSLRLSCRASGDVHKINILGWYRQAPAKEREMVAHITIGDATVYAESAKGRFTISRDEAKNMVYLQMNSLKPEDTAVYFCRAYSRIYPYNYWGQGTQVTVSS

SEQ ID NO: 16 - protein, 117 aa, synthetic construct
  REGION 1..117: note = Nanobody sequence
EVQLVESGGGLVQPGGSLRLSCAASGSVHLLNFLGWYRQCPGKEREMVAHITIADATDYSHFAKGRFTISRDEAKNMVYLQMNSLRPEDTAVYFCRAGSRIYPYDYWGQGTLVTVSS

SEQ ID NO: 17 - protein, 117 aa, synthetic construct
  REGION 1..117: note = Nanobody sequence
EVQLVESGGGLVQPGGSLRPSCAASGSVHLLNFLGWYRQAPGKEREMVAHITIADATDYAHFAKGRFTISRDEAKNMVYLQMNSLRPEDTAVYFCRAGSRIYPYDYWGQGTQVTVSS

SEQ ID NO: 18 - protein, 117 aa, synthetic construct
  REGION 1..117: note = Nanobody sequence
EVQLVESGGGLVQPGGSLRLSCAASGSVHLLNFLGWYRQAPGKEREMVAHITIADATDYAHFAKGRFTISRDEAKNMVYLQMNSLRPEDTAVYFCRAGSRIYPYDYWGQGTLVTVSS

SEQ ID NO: 19 - protein, 117 aa, synthetic construct
  REGION 1..117: note = Nanobody sequence
EVQLVESGGGLVQPGGSLKLSCAASGAVHKINFLGWYRQTPEKEREMVAHITIGDEVDYADSAKGRFTISRDEAKNMVYLQMTSLTPEDTAVYVCRAGSRLYPYNYWGQGTQVTVSS

SEQ ID NO: 20 - protein, 117 aa, synthetic construct
  REGION 1..117: note = Nanobody sequence
EVQLVESGGGLVHPGGSLRLSCAASGDVHKINFLGWHRQPPGKEREKVAHITIGDVTDYADSAKGRFTISRDEAKNMVYLQMNNLKPEDTAVYFCRAGSRIYPYDYWGQGTQVTVSS

SEQ ID NO: 21 - protein, 117 aa, synthetic construct
  REGION 1..117: note = Nanobody sequence
EVQLVESGGGLVQPGGSLRLSCAASGDVHKINVLGWYRQAPAKEREMVAHITIGDATDYADSAKGRFTISRDEAKNMVHLQMNSLKPEDTAVYFCRAYSRIYPYNYWGQGTQVTVSS

SEQ ID NO: 22 - protein, 117 aa, synthetic construct
  REGION 1..117: note = Nanobody sequence
EVQLVESGGGLVQPGGSLRLSCAASGDVHKINILGWYRQAPAKEREMVAHITIGDATNYADSAKGRFTISRDEAKNMVYLQMNSLKPEDTAVYFCRAYSRIYPYNYWGQGTLVTVSS

SEQ ID NO: 23 - protein, 117 aa, synthetic construct
  REGION 1..117: note = Nanobody sequence
EVQLVESGGGLVQPGGSLRLSCAASGDVHKINFLGWHRQAPGKEREKVAHITIGDVTDYADSAKGRFTISRDEAKNMVFLQMNNLKPEDTAVYFCRAGSRIYPYDYWGQGTQVTVSS

SEQ ID NO: 24 - protein, 117 aa, synthetic construct
  REGION 1..117: note = Nanobody sequence
EVQLVESGGGLVQPGGSLRLSCAASGDVHKINILGWYRQAPAKEREMVAHITIGDATDYAGSAKGRFTISRDEAKNMVYLQMNSLKPEDTAVYFCRAYSRIYPYNYWGQGTLVTVSS

SEQ ID NO: 25 - protein, 117 aa, synthetic construct
  REGION 1..117: note = Nanobody sequence
EVQLVESGGGLVQPGGSLRLSCAASGEVYKINFLGWYRQAPGKEREKVAHITIADVADYADFAKGRFTISRDEAKNMVYLQMNSLKPEDTAVYFCRAGSRIWPYDYWGQGTQVTVSS

SEQ ID NO: 26 - protein, 117 aa, synthetic construct
  REGION 1..117: note = Nanobody sequence
EVQLVESGGGLVQPGGSLKLSCAASGAVHKINFLGWYRQAPEKEREMVATITIGDEVDYADSAKGRFTISRDEAKNMVYLQMTSLKPEDTTVYVCRAGSRLYPYNYWGQGTQVTVSS

SEQ ID NO: 27 - protein, 117 aa, synthetic construct
  REGION 1..117: note = Nanobody sequence
EVQLVESGGGLVQPGGSLRLSCAASGEVYKINFLGWYRQAPGKEREKVAHITIADVADYADFAKGRFTISRDEAKNMVYLQMNSLKPEDTAVYFCRAGSRIWPYDYWGQGTLVTVSS

SEQ ID NO: 28 - protein, 117 aa, synthetic construct
  REGION 1..117: note = Nanobody sequence
EVQLVESGGGLVQPGGSLRLSCVASGDVHKINILGWYRQAPGKEREKVAHISISDQTDYAESAKGRFTISRDESKNMVYLQMNSLKPEDTAVYLCRAFSRIYPYDYWGQGTLVTVSS

SEQ ID NO: 29 - protein, 117 aa, synthetic construct
  REGION 1..117: note = Nanobody sequence
EVQLVESGGGLVQPGGSLRLSCAASGSVHKINFLGWYRQAPGKERELVATITIGDATDYADYAKGRFTISRDEARNMVYLQMNSLKPEDTAVYFCRAGSRLYPYNYWGQGTLVTVSS

SEQ ID NO: 30 - protein, 117 aa, synthetic construct
  REGION 1..117: note = Nanobody sequence
EVQLVESGGGLVQPGGSLRLSCAASGDVHKINILGWYRQAPAKEREMVAHITIGDATDYADSAKGRFAISRDEAKNMVYLQMNSLKPEDTAVYFCRAYSRIYPYNYWGQGTLVTVSS

SEQ ID NO: 31 - protein, 117 aa, synthetic construct
  REGION 1..117: note = Nanobody sequence
EVQLVESGGGLVQPGGSLRLSCAASGDVHKINFLGWHRQAPGKEREKVAHITIGDATDYADSAKGRFTISRDEAKNMVYLQMNSLKPEDTAVYFCRAGSRIYPYDYWGQGTQVTVSS

SEQ ID NO: 32 - protein, 117 aa, synthetic construct
  REGION 1..117: note = Nanobody sequence
EVQLVESGGGSVQPGGSLRLSCAASGSVHKINFLGWYRQAPGKEREVVATITIGDATDYADSAKGRFTISRDEAKNMVYLQMNSLSPEDTAVYFCRAGSRLYPYNYWGQGTQVTVSS

SEQ ID NO: 33 - protein, 117 aa, synthetic construct
  REGION 1..117: note = Nanobody sequence
EVQLVESGGGLVQPGGSARLSCVASGDVHKINFLGWYRQAPGKEREKVAHITIGDQTDYADSAKGRFTISRDEAKNMVYLQMNSLKPEDTAVYFCRAGSRIWPYDYWGQGTQVTVSS

SEQ ID NO: 34 - protein, 117 aa, synthetic construct
  REGION 1..117: note = Nanobody sequence
EVQLVESGGGLVQPGGSLRLSCAASGSVHLLNFLGWYRQAPGKEREMVAHITIADATDYSHFAKGRFTISRDEAKNMVYLQMNSLRPEDTAVYFCRAGSRIYPYDYWGQGTLVTVSS

SEQ ID NO: 35 - protein, 117 aa, synthetic construct
  REGION 1..117: note = Nanobody sequence
EVQLVESGGGLVQPGGSLRLSCAVSGSVHLLNFLGWYRQAPGKERGVVAHITIADATDYSHFAKGRFTISRDEAKNMVYLQMNSLRPEDTAVYFCRAGSRIYPYDYWGQGTQVTVSS

SEQ ID NO: 36 - protein, 117 aa, synthetic construct
  REGION 1..117: note = Nanobody sequence
EVQLVESGGGLVQAGGSLTLSCAASGDVHKINILGWYRQAPAKEREMVAHITIGDATDYADSAKGRFTISRDEAKNMVYLQMNSLKPEDTAVYFCRAYSRIYPYNYWGQGTLVTVSS

SEQ ID NO: 37 - protein, 117 aa, synthetic construct
  REGION 1..117: note = Nanobody sequence
EVQLVESGGGLVQPGGSLRLSCAASGGVHKINILGWYRQAPAKEREMVAHITIGDATDYADSAKGRFTISRDEAKNMVYLQMNSLKPEDTAVYFCRAYSRIYPYNYWGQGTLVTVSS

SEQ ID NO: 38 - protein, 117 aa, synthetic construct
  REGION 1..117: note = Nanobody sequence
EVQLVESGGGLVQPGGSLRLSCAASGEVYKINFLGWYRQAPGKEREKVAHITIADVADYADFAQGRFTISRDEAKNMVYLQMNSLKPEDTAVYFCRAGSRIWPYDYWGQGTQVTVSS

SEQ ID NO: 39 - protein, 117 aa, synthetic construct
  REGION 1..117: note = Nanobody sequence
EVQLVESGGGLVQPGGSLRLSCAASGDVHKINILGWYRQAPAKEREMVAHITIGDTTDYADSAKGRFTISRDEAKNMVYLQMNSLKPEDTAVYFCRAYSRIYPYNYWGQGTQVTVSS

SEQ ID NO: 40 - protein, 117 aa, synthetic construct
  REGION 1..117: note = Nanobody sequence
EVQLVESGGGLVQPGGSLRLSCAASGSVHLLNFLGWYRQAPGKEREMVAHITIADATDYSHFAKGRFTISRDEAKNMVYLQMNSLRPEDTAVYFCRAGSRIYPYDYWGHGTLVTVSS

SEQ ID NO: 41 - protein, 117 aa, synthetic construct
  REGION 1..117: note = Nanobody sequence
EVQLVESGGGLVQPGGSLRLSCVASGDVHKINFLGWYRQAPGKEREKVAHITIGDQADYADSAKGRFTISRDEAKNMVYLQMNSLKPEDTAVYFCRAGSRIYPYDYWGRGTLVTVSS

SEQ ID NO: 42 - protein, 117 aa, synthetic construct
  REGION 1..117: note = Nanobody sequence
EVQLVESGGGLVQPGGSLRLSCAVSGSVHLLNFLGWYRQAPGKEREMVTHITIADATDYSHFAKGRFTISRDEAKNMVYLQMNSLRPEDTAVYFCRAGSRIYPYDYWGQGTQVTVSS

SEQ ID NO: 43 - protein, 117 aa, synthetic construct
  REGION 1..117: note = Nanobody sequence
EVQLVESGGDLVQPGGSLRLSCAASGDVHKINFLGWYRQAPGKEREMVAHITIADATDYAEFAKGRFTISRDEPKNMVHLQMNSLKPEDTAVYLCRAGSRIYPYNYWGQGTQVTVSS

SEQ ID NO: 44 - protein, 117 aa, synthetic construct
  REGION 1..117: note = Nanobody sequence
EVQLVESGGGLVQPGGSLRLSCAASGDVHKINILGWYRQAPAKEREMVAHITIGDATDYADSAKGRFTISRDEAKNMVYLQMNSLKPEDTAVYFCRAYSRIYPYNYWGRGTQVTVSS

SEQ ID NO: 45 - protein, 117 aa, synthetic construct
  REGION 1..117: note = Nanobody sequence
EVQLVESGGGLVQPGGSLRLSCVASGDVHKINILGWYRQAPGKEREKVARISISDQTDYAESAKGRFTISRDESKNMVYLQMNSLKPEDTAVYLCRAFSRIYPYDYWGQGTLVTVSS

SEQ ID NO: 46 - protein, 117 aa, synthetic construct
  REGION 1..117: note = Nanobody sequence
EVQLVESGGGLVQPEGSLRLSCAASGEVYKINFLGWYRQAPGKEREKVAHITIADVADYADFAKGRLTISRDEAKNMVYLQMNSLKPEDTAVYFCRAGSRIWPYDYWGQGTLVTVSS

SEQ ID NO: 47 - protein, 117 aa, synthetic construct
  REGION 1..117: note = Nanobody sequence
EVQLVESGGGLVQPGGSLKLPCAASGAVHKINFLGWYRQTPEKEREMVATITIGDEVDYADSAKGRFTISRDEAKNMVYLQMTSLKPEDTAVYVCRAGSRLYPYNYWGQGTLVTVSS

SEQ ID NO: 48 - protein, 117 aa, synthetic construct
  REGION 1..117: note = Nanobody sequence
EVQLVESGGGLVQPGGSLGLSCAASGSVHLLNFLGWYRQAPGKEREMVAHITIADATDYAHFAKGRFTISRDEAKNMVYLQMNSLRPEDTAVYFCRAGSRIYPYDYWGQGTLVTVSS

SEQ ID NO: 49 - protein, 117 aa, synthetic construct
  REGION 1..117: note = Nanobody sequence
EVQLVESGGGLAQPGGSLRLSCAASGDVHKINILGWYRQAPAKEREMVAHITIGDATDYADSAKGRFTISRDEAKNMVYLQMNSLKPEDTAVYFCRAYSRIYPYNYWGQGTLVTVSS

SEQ ID NO: 50 - protein, 117 aa, synthetic construct
  REGION 1..117: note = Nanobody sequence
EVQLVESGGGLVQPGGSLRLSCVASGDVHKINFLGWYRQAPGKEREKVAHISIGDQTDYADSAKGRFTISRDESKNMVYLQMNSLKPEDTAVYFCRAFSRIYPYDYWGQGTLVTVSS

SEQ ID NO: 51 - protein, 117 aa, synthetic construct
  REGION 1..117: note = Nanobody sequence
EVQLVESGGGLVQPGGSLRLSCAASGEVYKINFLGWYRQAPGKEREKVAHITIADAADYADFAKGRFTISRDGAKNMVYLQMNSLKPEDTAVYFCRAGSRIWPYDYWGQGTQVTVSS

SEQ ID NO: 52 - protein, 117 aa, synthetic construct
  REGION 1..117: note = Nanobody sequence
EVQLVESGGGWVQPGGSLRLSCAASGSVYKINFLSWYRQAPGHERELVATITIGDAADYADSAKGRFTISRDEARNMVYLQMNSLKPEDTALYFCHAGSRLYPYNYWGQGTQVTVSS

SEQ ID NO: 53 - protein, 117 aa, synthetic construct
  REGION 1..117: note = Nanobody sequence
EVQLVESGGGLVQPGGSLRLSCAASGSVHLLNFLGWYRQAPGKEREMVAHITIADATDYSHFAKGRFTISRDEAKNMVYLQMNSLRPEDTAVYFCRAGSRIYPYDYWGQGTQVTVSS

SEQ ID NO: 54 - protein, 117 aa, synthetic construct
  REGION 1..117: note = Nanobody sequence
EVQLVESGGGLVQPGGSLRLSCVASGDVHKINILGWYRQAPGKEREKVAHIAISDQTDYAESAKGRFTISRDESKNMVYLQMNSLKPEDTAVYLCRAFSRIYPYDYWGQGTLVTVSS

SEQ ID NO: 55 - protein, 117 aa, synthetic construct
  REGION 1..117: note = Nanobody sequence
EVQLVESGGGLVQPGGSLRLSCAASGDVHKINILGWYRQAPAKEREMVAHITIGDATDYADSAKGRFTISRDEAKNMVYLQMNSLKPEDTAAYFCRAYSRIYPYNYWGQGTLVTVSS

SEQ ID NO: 56 - protein, 117 aa, synthetic construct
  REGION 1..117: note = Nanobody sequence
EVQLVESGGGLVQPGGSLRLSCAASGDVHKINILGWYRQAPAKERGMVAHITIGDATDYADSAKGRFTISRDEAKNMVYLQMNSLKPEDTAVYFCRAYSRIYPYNYWGQGTQVTVSS

SEQ ID NO: 57 - protein, 117 aa, synthetic construct
  REGION 1..117: note = Nanobody sequence
EVQLVESGGGLVQPGGSLRLSCAASGDVHKINILGWYRQAPAKEHEMVAHITIGDATDYADSAKGRFTISRDEAKNMVYLQMNSLKPEDTAVYFCRAYSRIYPYNYWGQGTLVTVSS

SEQ ID NO: 58 - protein, 117 aa, synthetic construct
  REGION 1..117: note = Nanobody sequence
EVQLVESGGGLVQPGGSLRLSCAASGDVHKINILGWYRQAPAREREMVAHITIGDATDYADSAKGRFTISRDEAKNMVYLQMNSLKPEDTAVYFCRAYSRIYPYNYWGQGTQVTVSS

SEQ ID NO: 59 - protein, 117 aa, synthetic construct
  REGION 1..117: note = Nanobody sequence
EVQLVESGGGLVQPGGSLRLSCAASGDVHKINILGWYRQAPAKEREMVAHITIGDATDYADSAKGRFTISRDEAENMVYLQMNSLKPEDTAVYFCRAYSRIYPYNYWGQGTLVTVSS

SEQ ID NO: 60 - protein, 117 aa, synthetic construct
  REGION 1..117: note = Nanobody sequence
EVQLVESGGGLVQPGGSLKLSCAASGAVHKINFLGWYRQTPEKEREMVATITIGDEVDYADSAKGRFTISRDEAKNMVYLQMTSLKPEDTAVYVCRAGSRLYPYNYWGQGTLVTVSS

SEQ ID NO: 61 - protein, 117 aa, synthetic construct
  REGION 1..117: note = Nanobody sequence
EVQLVESGGGLVQPGGSLKLSCAASGAVHKINFLGWYRQAPEKEREMVATITIGDEVDYADSAKGRFTISRDEATNMVYLQMTSLKPEDTAVYFCRAGSRIYPYNYWGQGTQVTVSS

SEQ ID NO: 62 - protein, 117 aa, synthetic construct
  REGION 1..117: note = Nanobody sequence
EVQLVESGGGLVQPGGSLRLSCAASGDVHKINILGWYRQAPAKEREMVAHITIGDATSYAGSAKGRFTISRDEAKNMVYLQLNNLKPEDTAVYFCRAYSRIYPYNYWGQGTLVTVSS

SEQ ID NO: 63 - protein, 117 aa, synthetic construct
  REGION 1..117: note = Nanobody sequence
EVQLVESGGGLVQPGGSLRLSCAASGDVHKINILGWYRQAPAKEREMVAHITIGDATSYADSAKGRFTISRDEAKNMVYLQLNNLKPEDTAVYFCRAYSRIYPYNYWGQGTLVTVSS

SEQ ID NO: 64 - protein, 117 aa, synthetic construct
  REGION 1..117: note = Nanobody sequence
EVQLVESGGDLVQPGGSLRLSCAASGDVHKINFLGWYRQAPGKEREMVAHITIADATDYAEFAKGRFTISRDEPKNMVYLQMNSLKPEDTAVYLCRAGSRIYPYNYWGQGTQVTVSS

SEQ ID NO: 65 - protein, 117 aa, synthetic construct
  REGION 1..117: note = Nanobody sequence
EVQLVESGGGLVQPGGSLKLSCAASGAVHKINFLGWYRQTPEKEREMVATITIGDEVDYAHSAKGRFTISRDEAKNMVYLQMTSLKPEDTAVYVCRAGSRLYPYNYWGQGTQVTVSS

SEQ ID NO: 66 - protein, 117 aa, synthetic construct
  REGION 1..117: note = Nanobody sequence
EVQLVESGGGLVQPGGSLKLSCAASGAVHKINFLGWYRQTPEKEREMVATITIGDEVAYADSAKGRFTISRDEAKNMVYLQMTSLKPEDTAVYVCRAGSRLYPYNYWGQGTQVTVSS

SEQ ID NO: 67 - protein, 117 aa, synthetic construct
  REGION 1..117: note = Nanobody sequence
EVQLVESGGGLVQPGGSLRLSCAASGEVYKINFLGWYRQAPGKEREKVAHITIADAADYADFAKGRFTISRDEAKNMVYLQMNSLKPEDTAVYFCRAGSRIWPYDYWGQGTQVTVSS

SEQ ID NO: 68 - protein, 117 aa, synthetic construct
  REGION 1..117: note = Nanobody sequence
EVQLVESGGGLVQPGGSLRLSCAASGEVYKINFLGWYRQAPGKEREKVAHITIADAADYADFAKGRFTISRDEAKNMVYLQMNSLKPEDTAVYFCRAGSRIYPYDYWGQGTQVTVSS

SEQ ID NO: 69 - protein, 117 aa, synthetic construct
  REGION 1..117: note = Nanobody sequence
EVQLVESGGGSVQPGGSLRPSCAASGSVHKINFLGWYRQAPGKEREMVATITIGDATDYADSAKGRFTISRDEAKNMVYLQMNSLSPEDTAVYFCRAGSRLYPYNYWGQGTQVTVSS

SEQ ID NO: 70 - protein, 117 aa, synthetic construct
  REGION 1..117: note = Nanobody sequence
EVQLVESGGGLVQPGGSLRLSCAASGEVYKINFLGWYRQAPGKEREKVAHITIADVADYADFAKGRFTISRDEVKNMVYLQMNSLKPEDTAVYFCRAGSRIWPYDYWGQGTLVTVSS

SEQ ID NO: 71 - protein, 117 aa, synthetic construct
  REGION 1..117: note = Nanobody sequence
EVQLVESGGGLVQPGESLRLSCAASGDVHKINILGWYRQAPAKEREMVAHITIGDATDYADSAKGRFTISRDEAKNMVYLQMNSLKPEDTAVYFCRAYSRIYPYNYWGQGTLVTVSS

SEQ ID NO: 72 - protein, 117 aa, synthetic construct
  REGION 1..117: note = Nanobody sequence
EVQLVESGGGLVQPGGSLRLSCAASGEVYKINFLGWYRQAPGKEREKVAHITIADAADYADFAKGRFTISRDEAKNMVYLQMNSLRPEDTAVYFCRAGSRIWPYDYWGQGTQVTVSS

SEQ ID NO: 73 - protein, 117 aa, synthetic construct
  REGION 1..117: note = Nanobody sequence
EVQLVESGGGLVQPGGSLRLSCAASGSVHLLNFLGWYRQAPGKEREMVAHITIADVTDYSYFAKGRFTISRDEAKNMVYLQMNSLRPEDTAVYFCRAGSRIYPYDYWGQGTQVTVSS

SEQ ID NO: 74 - protein, 117 aa, synthetic construct
  REGION 1..117: note = Nanobody sequence
EVQLVESGGGLVQPGGSLRLSCAASGDVHKINILGWYRQAPAKEREMVAHITIGDATDYADSAKGRFTISRDEAKNVVYLQMNSLKPEDTAVYFCRAYSRIYPYNYWGQGTLVTVSS

SEQ ID NO: 75 - protein, 117 aa, synthetic construct
  REGION 1..117: note = Nanobody sequence
EVQLVESGGGSVQPGGSLRLSCAASGSVHKINFLGWYRQAPGKERGMVATITIGDATDYADSAKGRFTISRDEAKNMVYLQMNSLSPEDTAVYFCRAGSRLYPYNYWGQGTQVTVSS

SEQ ID NO: 76 - protein, 117 aa, synthetic construct
  REGION 1..117: note = Nanobody sequence
EVQLVESGGGLVQPGGSLKLSCAASGAVHKINFLGWYRQTPEKEREMVATITIGDEVDYEDSAKGRFTISRDEAKNMVYLQMTGLKPEDTAVYVCRAGSRLYPYNYWGQGTLVTVSS

SEQ ID NO: 77 - protein, 117 aa, synthetic construct
  REGION 1..117: note = Nanobody sequence
EVQLVESGGGLVRPGGSLRLSCVASGDVHKINILGWYRQAPGKEREKVAHISISDQTDYAESAKGRFTISRDESKNMVYLQMNSLKPEDTAVYLCRAFSRIYPYDYWGQGTQVTVSS

SEQ ID NO: 78 - protein, 117 aa, synthetic construct
  REGION 1..117: note = Nanobody sequence
EVQLVESGGGLVQPGGSLRLSCAASGDVYKINFLGWHRQAPGKEREKVAHITIGDATDYADSAKGRFTISRDEAKNMVYLQMNSLKPEDTAVYFCRAGSRIYPYDYWGQGTLVTVSS

SEQ ID NO: 79 - protein, 117 aa, synthetic construct
  REGION 1..117: note = Nanobody sequence
EVQLVESGGGLVQPGGSLRLSCRASGDVHKINILGWYRQAPAKEREMIAHITIGDATDYAESAKGRFTISRDEAKNMVYLQMNSLKPEDTAVYFCRAYSRIYPYNYWGQGTQVTVSS

SEQ ID NO: 80 - protein, 117 aa, synthetic construct
  REGION 1..117: note = Nanobody sequence
EVQLVESGGGLVQPGGSLRLSCAASGDVHKINILGWYRQAPAKGREMVAHITIGDATDYADSAKGRFTISRDEAKNMVYLQMNSLKPEDTAVYFCRAYSRIYPYNYWGQGTQVTVSS

SEQ ID NO: 81 - protein, 117 aa, synthetic construct
  REGION 1..117: note = Nanobody sequence
EVQLVESGGDLVQPGGSLRLSCAASGDVHKINFLGWYRQAPGKEREMVAHITIADATDYAEFAKGRFTISRDEPKNMVYLQMNSLKPEDTAVYLCRAGSRIYPYSYWGQGTQVTVSS

SEQ ID NO: 82 - protein, 117 aa, synthetic construct
  REGION 1..117: note = Nanobody sequence
EVQLVESGGGMVQPGGSLRLSCAASGDVHKINILGWYRQAPAKEREMVAHITIGDATDYADSAKGRFTISRDEAKNMVYLQMNSLKPEDTAVYFCRAYSRIYPYNYWGQGTLVTVSS

SEQ ID NO: 83 - protein, 117 aa, synthetic construct
  REGION 1..117: note = Nanobody sequence
EVQLVESGGGLVQPGGSLRLSCAASGDVHKINILGWYRQVPAKEREMVAHITIGDATDYADSAKGRFTISRDEAKNMVYLQMNSLKPEDTAAYFCRAYSRIYPYNYWGQGTLVTVSS

SEQ ID NO: 84 - protein, 117 aa, synthetic construct
  REGION 1..117: note = Nanobody sequence
EVQLVESGGGLVQPGGSLRLSCAASGEVYKINFLGWYRQAPGKEREKVAHITIADAADYADFAKGRFTISRDEAKNMVYLQMNSLKPEDTAVYFCRAGSRIWPYDYWGQGTLVTVSS

SEQ ID NO: 85 - protein, 117 aa, synthetic construct
  REGION 1..117: note = Nanobody sequence
EVQLVESGGGLVQPGGSLRLSCAASGSVHLLNFLGWYRQAPGKEREMVAHITIADATDYSHFAKGRFTISRDEAKNMVYLQMNGLRPEDTAVYFCRAGSRIYPYDYWGQGTLVTVSS

SEQ ID NO: 86 - protein, 117 aa, synthetic construct
  REGION 1..117: note = Nanobody sequence
EVQLVESGGGLVQPGGSLRLSCAASGDVHKINFLGWYRQAPGKEREMVAHITIADATDYAEFAKGRFTISRDEPKNMVYLQMNSLKPEDTAVYLCRAGSRIYPYNYWGQGTQVTVSS

SEQ ID NO: 87 - protein, 117 aa, synthetic construct
  REGION 1..117: note = Nanobody sequence
EVQLVESGGGLVQPGGSLRLSCAASGEVHKINILGWYRQCPGKERDMVATITIGDATDYADSAKGRFTISRDEAKNMVYLQMNSLKPEDTAVYFCRALSRLYPYNYWGQGTLVTVSS

SEQ ID NO: 88 - protein, 117 aa, synthetic construct
  REGION 1..117: note = Nanobody sequence
EVQLVESGGGLVQPGGSLRLSCAASGDVHKINILGWYRQAPAKEREMVAHITIGDATDYADSAKGRFTISRDEAKNMVYLQMNSLKPEDTAVYLCRAYSRIYPYNYWGQGTQVTVSS

SEQ ID NO: 89 - protein, 117 aa, synthetic construct
  REGION 1..117: note = Nanobody sequence
EVQLVESGGGLVQPGGSLRLSCAASGEVYKINFLGWQRQAPGKEREKVAHITIADVADYADFAKGRFTISRDEAKNMVYLQMNSLKPEDTAVYFCRAGSRIWPYDYWGQGTLVTVSS

SEQ ID NO: 90 - protein, 117 aa, synthetic construct
  REGION 1..117: note = Nanobody sequence
EVQLVESGGDLVQPGGSLRLSCAASGDVHKINFLGWYRQAPGKEREMVAHITIADATDYAEFAKGRFTISRDEPKNMVYLQMNSLKPVDTAVYLCRAGSRIYPYNYWGQGTLVTVSS

SEQ ID NO: 91 - protein, 117 aa, synthetic construct
  REGION 1..117: note = Nanobody sequence
EVQLVESGGGLVQPGGSLRLSCAASGSVHLLNFLGWYRQAPGKEREKVAHITIADATDYSHFAKGRFTISRDEAKNMVYLQMNNLRPEDTAVYFCRAGSRIYPYDYWGQGTLVTVSS

SEQ ID NO: 92 - protein, 117 aa, synthetic construct
  REGION 1..117: note = Nanobody sequence
EVQLVESGGGLVQPGGSPRLSCVASGDVHKINFLGWYRQAPGKEREKVAHITIGDQADYADSAKGRFTISRDEAKNMVYLQMNSLKPEDTAVYFCRAGSRIYPYDYWGQGTLVTVSS

SEQ ID NO: 93 - protein, 117 aa, synthetic construct
  REGION 1..117: note = Nanobody sequence
EVQLVESGGGLVQPGGSLRLSCAASGDVHKINILGWYRQAPAKEREMVAHITIGDATDYADSAKGRFTISRDEAKNMVYLQMNSLKPEDAAVYFCRAYSRIYPYNYWGQGTLVTVSS

SEQ ID NO: 94 - protein, 117 aa, synthetic construct
  REGION 1..117: note = Nanobody sequence
EVQLVESGGGLVQPGGSLRLSCAASGEVYKINFLGWYRQAPGKEREKVAHITIADVADYADFAKGRFTISRDGAKNMVYLQMNSLKPEDTAVYFCRAGSRIWPYDYWGQGTLVTVSS

SEQ ID NO: 95 - protein, 117 aa, synthetic construct
  REGION 1..117: note = Nanobody sequence
EVQLVESGGGSVQPGGSLRLSCAASGSVHKINFLGWYCQAPGKEREMVATITIGDATDYADSAKGRFTISRDEAKNMVYLQMNSLSPEDTAVYFCRAGSRLYPYNYWGQGTQVTVSS

SEQ ID NO: 96 - protein, 117 aa, synthetic construct
  REGION 1..117: note = Nanobody sequence
EVQLVESGGGLVQPGGSLRLSCVASGDVHKINILGWYRQAPGKEREKVAHISISDQTDYAESAKGRFTISRDESKNMVYLQMNSLKPEDAAVYLCRAFSRIYPYDYWGQGTQVTVSS

SEQ ID NO: 97 - protein, 117 aa, synthetic construct
  REGION 1..117: note = Nanobody sequence
EVQLVESGGGLVQPGGSLRPSCAASGEVYKINFLGWYRQAPGKEREKVAHITIADVADYADFAKGRFTISRDEAKNMVYLQMNSLKPEDTAVYFCRAGSRIWPYDYWGQGTQVTVSS

SEQ ID NO: 98 - protein, 117 aa, synthetic construct
  REGION 1..117: note = Nanobody sequence
EVQLVESGGGLVQPGGSLRPSCVASGDVHKINFLGWYRQAPGKEREKVAHITIADQADYADSAKGRFTISRDEAKNMVYLQMNSLKPEDTAVYFCRAGSRIYPYDYWGQGTLVTVSS

SEQ ID NO: 99 - protein, 117 aa, synthetic construct
  REGION 1..117: note = Nanobody sequence
EVQLVESGGGLVQPGGSLRLSCAASGEVHKINILGWYRQAPGKERDMVATITIGDETQYADSAKGRFTISRDEAKNMVYLQMNSLKPEDTAVYFCRALSRLYPYNYWGQGTLVTVSS

SEQ ID NO: 100 - protein, 117 aa, synthetic construct
  REGION 1..117: note = Nanobody sequence
EVQLVESGGGLVQPGGSLRLSCAASGDVHKINILGWYRQAPAKEREMVAHITIGDATDYADSAKGRFTISRDEAKNMVYLQMDSLKPEDTAVYFCRAYSRIYPYNYWGQGTLVTVSS

SEQ ID NO: 101 - protein, 117 aa, synthetic construct
  REGION 1..117: note = Nanobody sequence
EVQLVESGGGLVQPGGSLRLSCAASGDVHKINILGWYRQAPAKEREMVAHITIGDATDYADSAKGRFTISRDEAKNMVYLQMNSLKPGDTAVYFCRAYSRIYPYNYWGQGTLVTVSS

SEQ ID NO: 102 - protein, 117 aa, synthetic construct
  REGION 1..117: note = Nanobody sequence
EVQLVESGGGLVQPGGSLRLSCAASGDVHKINILGWHRQAPAKEREMVAHITIGDATDYADSAKGRFTISRDEAKNMVYLQMNSLKPEDTAVYFCRAYSRIYPYNYWGQGTLVTVSS

SEQ ID NO: 103 - protein, 117 aa, synthetic construct
  REGION 1..117: note = Nanobody sequence
EVQLVESGGGLVQPGGSLRLSCAASGDVHKINILGWHRQAPAKEREMVAHITIGDATDYADSAKGRFTISRDEAKNMVYLQMNSLKPEDTAAYFCRAYSRIYPYNYWGQGTQVTVSS

SEQ ID NO: 104 - protein, 117 aa, synthetic construct
  REGION 1..117: note = Nanobody sequence
EVQLVESGGGWVQAGGSLRLSCAASGDVHKINILGWYRQAPAKEREMVAHITIGDATDYADSAKGRFTISRDEAKNMVYLQMNSLKPEDTAVYFCRAYSRIYPYNYWGQGTLVTVSS

SEQ ID NO: 105 - protein, 117 aa, synthetic construct
  REGION 1..117: note = Nanobody sequence
EVQLVESGGGLVQPGGSLRLSCITSGETFKINIWGWYRQAPGKQRELVASLTIGGATDYADSVKGRFTISEDSAKNTVYLQMNSLKAEDTAVYFCNAKSRLYPYDYWGQGTQVTVSS

SEQ ID NO: 106 - protein, 117 aa, synthetic construct
  REGION 1..117: note = Nanobody sequence
EVQLVESGGGLVQPGGSLRLSCITSGETFKINIWGWYRQAPGKQRELVASLTIGGATNYADSVKGRFTISEDSAKNTVYLQMNSLKPEDTAVYFCNAKSRLYPYDYWGQGTLVTVSS

SEQ ID NO: 107 - protein, 117 aa, synthetic construct
  REGION 1..117: note = Nanobody sequence
EVQLVESGGGLVQPGGSLRLSCITSGETFKINIWGWYRQAPGKRRELVASLTIGGATNYADSVKGRFTISEDSAKNTVYLQMNSLKPEDTAVYFCNAKSRIYPYDYWGQGTQVTVSS

SEQ ID NO: 108 - protein, 117 aa, synthetic construct
  REGION 1..117: note = Nanobody sequence
EVQLVESGGGLVQPGGSLRLSCITSGETFKINIWGWYRQTPGKQRELVASLTIGGATNYADSVKGRFTISEDSAKNTVYLQMNSLKPEDTAVYFCNAKSRLYPYDYWGQGTQVTVSS

SEQ ID NO: 109 - protein, 117 aa, synthetic construct
  REGION 1..117: note = Nanobody sequence
EVQLVESGGGLVQPGGSLRLSCITSGQTFKINIWGWYRQAPGKQRELVASLTIGGATNYADSVKGRFTISEDSAKNTVYLQMNSLKPEDTAVYFCNAKSRLYPYDYWGQGTQVTVSS

SEQ ID NO: 110 - protein, 117 aa, synthetic construct
  REGION 1..117: note = Nanobody sequence
EVQLVESGGGLVQPGGSLRLSCITSGETFKVNIWGWYRQGPGKQRELVASLTIGGATNYADSVKGRFTISEDSAKNTVYLQMNSLKPEDTAVYFCNAKSRLYPYDYWGRGTQVTVSS

SEQ ID NO: 111 - protein, 118 aa, synthetic construct
  REGION 1..118: note = Nanobody sequence
EVQLVEESGGGLVQPGGSLRLSCITSGETFKINIWGWYRQAPGKQRELVASLTIGGATNYADSVKGRFTISEDSAKNTVYLQMNSLKPEDTAVYFCNAKSRIYPYDYWGRGTQVTVSS

SEQ ID NO: 112 - protein, 117 aa, synthetic construct
  REGION 1..117: note = Nanobody sequence
EVQLVESGGGLVQPGGSLRLSCITSGETFKINIWGWYRQAPGKQRELVASLTIGGATNYADSVKGRFTISEDSAKNTVYLQMNSLKPEDTAVYFCNAKSRLYPYDYWDQGTQVTVSS

SEQ ID NO: 113 - protein, 117 aa, synthetic construct
  REGION 1..117: note = Nanobody sequence
EVQLVESGGGLVQPGGSLRLSCLTSGETFKVNIWGWYRQGPGKQRELVASLTIGGATNYADSVKGRFTISEDSAKNTVYLQMSSLKPEDTAVYFCNAKSRLYPYDYWGQGTQVTVSS

SEQ ID NO: 114 - protein, 117 aa, synthetic construct
  REGION 1..117: note = Nanobody sequence
EVQLVESGGGLVQPGGSLRLSCITSGETFKINIWGWYRQAPGKQRELVASLTIGGATNYADSVKGRFTISEDSAKNTVYLQMNSLKPEDTAVYFCNAKSRIYPYDYWGRGTQVTVSS

SEQ ID NO: 115 - protein, 117 aa, synthetic construct
  REGION 1..117: note = Nanobody sequence
EVQLVESGGGLVQPGGSLRLSCITSGETFKINIWGWYRQAPGKQRELVASLTIGGATNYADSVKGRFTISEDSAKDTVYLQMNSLKPEDTAVYFCNAKSRLYPYDYWGQGTLVTVSS

SEQ ID NO: 116 - protein, 117 aa, synthetic construct
  REGION 1..117: note = Nanobody sequence
EVQLVESGGGLVQPGGSLRLSCAASGEIGRINFYRWYRQAPGNQREVVATITIADKTDYADSAKGRFTISRDESRNMVYLQMSSLKPEDTAVYFCHAGSRLYPYDYWGQGTQVTVSS

SEQ ID NO: 117 - protein, 117 aa, synthetic construct
  REGION 1..117: note = Nanobody sequence
EVQLVESGGGLVQPGGSLRLSCAASGEIGRINFYRWYRQAPGNQRGVVATITIADKIDYADSAKGRFTISRDESRNMVYLQMGSLKPEDTAVYFCHAGSRLYPYDYWGQGTQVTVSS

SEQ ID NO: 118 - protein, 117 aa, synthetic construct
  REGION 1..117: note = Nanobody sequence
EVQLVESGGGLVQPGGSLRLSCAASGEIGRINFYRWYRQAPGNQREVVATITIADKTDYADSAKGRFTISRDESRNMVYLQMSSLKPENTAVYFCHAGSRLYPYDYWGQGTQVTVSS

SEQ ID NO: 119 - protein, 10 aa, synthetic construct
  REGION 1..10: note = CDR1
GSVHKINFLG

SEQ ID NO: 120 - protein, 10 aa, synthetic construct
  REGION 1..10: note = CDR1
GSVHLLNFLG

SEQ ID NO: 121 - protein, 10 aa, synthetic construct
  REGION 1..10: note = CDR1
GAVHKINFLG

SEQ ID NO: 122 - protein, 10 aa, synthetic construct
  REGION 1..10: note = CDR1
GDVHKINILG

SEQ ID NO: 123 - protein, 10 aa, synthetic construct
  REGION 1..10: note = CDR1
GDVHKINFLG

SEQ ID NO: 124 - protein, 10 aa, synthetic construct
  REGION 1..10: note = CDR1
GETFKINIWG

SEQ ID NO: 125 - protein, 10 aa, synthetic construct
  REGION 1..10: note = CDR1
GDVHKINVLG

SEQ ID NO: 126 - protein, 10 aa, synthetic construct
  REGION 1..10: note = CDR1
GEVYKINFLG

SEQ ID NO: 127 - protein, 10 aa, synthetic construct
  REGION 1..10: note = CDR1
GGVHKINILG

SEQ ID NO: 128 - protein, 10 aa, synthetic construct
  REGION 1..10: note = CDR1
GQTFKINIWG

SEQ ID NO: 129 - protein, 10 aa, synthetic construct
  REGION 1..10: note = CDR1
GSVYKINFLS

SEQ ID NO: 130 - protein, 10 aa, synthetic construct
  REGION 1..10: note = CDR1
GEIGRINFYR

SEQ ID NO: 131 - protein, 10 aa, synthetic construct
  REGION 1..10: note = CDR1
GETFKVNIWG

SEQ ID NO: 132 - protein, 10 aa, synthetic construct
  REGION 1..10: note = CDR1
GDVYKINFLG

SEQ ID NO: 133 - protein, 10 aa, synthetic construct
  REGION 1..10: note = CDR1
GEVHKINILG

SEQ ID NO: 134 - protein, 9 aa, synthetic construct
  REGION 1..9: note = CDR2
TITIGDTTD

SEQ ID NO: 135 - protein, 9 aa, synthetic construct
  REGION 1..9: note = CDR2
TITIGDATD

SEQ ID NO: 136 - protein, 9 aa, synthetic construct
  REGION 1..9: note = CDR2
HITIADATD

SEQ ID NO: 137 - protein, 9 aa, synthetic construct
  REGION 1..9: note = CDR2
TITIGDDVD

SEQ ID NO: 138 - protein, 9 aa, synthetic construct
  REGION 1..9: note = CDR2
HITIGDATD

SEQ ID NO: 139 - protein, 9 aa, synthetic construct
  REGION 1..9: note = CDR2
HITIGDQAD

SEQ ID NO: 140 - protein, 9 aa, synthetic construct
  REGION 1..9: note = CDR2
HISIADATD

SEQ ID NO: 141 - protein, 9 aa, synthetic construct
  REGION 1..9: note = CDR2
HITIGDATV

SEQ ID NO: 142 - protein, 9 aa, synthetic construct
  REGION 1..9: note = CDR2
SLTIGGATD

SEQ ID NO: 143 - protein, 9 aa, synthetic construct
  REGION 1..9: note = CDR2
HITIGDEVD

SEQ ID NO: 144 - protein, 9 aa, synthetic construct
  REGION 1..9: note = CDR2
HITIGDVTD

SEQ ID NO: 145 - protein, 9 aa, synthetic construct
  REGION 1..9: note = CDR2
SLTIGGATN

SEQ ID NO: 146 - protein, 9 aa, synthetic construct
  REGION 1..9: note = CDR2
HITIGDATN

SEQ ID NO: 147 - protein, 9 aa, synthetic construct
  REGION 1..9: note = CDR2
HITIADVAD

SEQ ID NO: 148 - protein, 9 aa, synthetic construct
  REGION 1..9: note = CDR2
TITIGDEVD

SEQ ID NO: 149 - protein, 9 aa, synthetic construct
  REGION 1..9: note = CDR2
HISISDQTD

SEQ ID NO: 150 - protein, 9 aa, synthetic construct
  REGION 1..9: note = CDR2
HITIGDQTD

SEQ ID NO: 151 - protein, 9 aa, synthetic construct
  REGION 1..9: note = CDR2
HITIGDTTD

SEQ ID NO: 152 - protein, 9 aa, synthetic construct
  REGION 1..9: note = CDR2
RISISDQTD

SEQ ID NO: 153 - protein, 9 aa, synthetic construct
  REGION 1..9: note = CDR2
HISIGDQTD

SEQ ID NO: 154 - protein, 9 aa, synthetic construct
  REGION 1..9: note = CDR2
HITIADAAD

SEQ ID NO: 155 - protein, 9 aa, synthetic construct
  REGION 1..9: note = CDR2
TITIGDAAD

SEQ ID NO: 156 - protein, 9 aa, synthetic construct
  REGION 1..9: note = CDR2
HIAISDQTD

SEQ ID NO: 157 - protein, 9 aa, synthetic construct
  REGION 1..9: note = CDR2
TITIADKTD

SEQ ID NO: 158 - protein, 9 aa, synthetic construct
  REGION 1..9: note = CDR2
TITIADKID

SEQ ID NO: 159 - protein, 9 aa, synthetic construct
  REGION 1..9: note = CDR2
HITIGDATS

SEQ ID NO: 160 - protein, 9 aa, synthetic construct
  REGION 1..9: note = CDR2
TITIGDEVA

SEQ ID NO: 161 - protein, 9 aa, synthetic construct
  REGION 1..9: note = CDR2
HITIADVTD

SEQ ID NO: 162 - protein, 9 aa, synthetic construct
  REGION 1..9: note = CDR2
HITIADQAD

SEQ ID NO: 163 - protein, 9 aa, synthetic construct
  REGION 1..9: note = CDR2
TITIGDETQ

SEQ ID NO: 164 - protein, 9 aa, synthetic construct
  REGION 1..9: note = CDR3
GSRLYPYNY

SEQ ID NO: 165 - protein, 9 aa, synthetic construct
  REGION 1..9: note = CDR3
GSRIYPYDY

SEQ ID NO: 166 - protein, 9 aa, synthetic construct
  REGION 1..9: note = CDR3
YSRIYPYNY

SEQ ID NO: 167 - protein, 9 aa, synthetic construct
  REGION 1..9: note = CDR3
KSRLYPYDY

SEQ ID NO: 168 - protein, 9 aa, synthetic construct
  REGION 1..9: note = CDR3
KSRIYPYDY

SEQ ID NO: 169 - protein, 9 aa, synthetic construct
  REGION 1..9: note = CDR3
GSRIWPYDY

SEQ ID NO: 170 - protein, 9 aa, synthetic construct
  REGION 1..9: note = CDR3
FSRIYPYDY

SEQ ID NO: 171 - protein, 9 aa, synthetic construct
  REGION 1..9: note = CDR3
GSRIYPYNY

SEQ ID NO: 172 - protein, 9 aa, synthetic construct
  REGION 1..9: note = CDR3
GSRLYPYDY

SEQ ID NO: 173 - protein, 9 aa, synthetic construct
  REGION 1..9: note = CDR3
GSRIYPYSY

SEQ ID NO: 174 - protein, 9 aa, synthetic construct
  REGION 1..9: note = CDR3
LSRLYPYNY

SEQ ID NO: 175 - protein, 25 aa, synthetic construct [sequence omitted]

SEQ ID NO: 176 - protein, 25 aa, synthetic construct
  REGION 1..25: note = FR1
EVQLVESGGGLVQPGRSLRLPCAAS

SEQ ID NO: 177 - protein, 25 aa, synthetic construct [sequence omitted]

SEQ ID NO: 178 - protein, 25 aa, synthetic construct
  REGION 1..25: note = FR1
EVQLVESGGGLVQPGGSLKLSCAAS

SEQ ID NO: 179 - protein, 25 aa, synthetic construct
  REGION 1..25: note = FR1
EVQLVESGGGLVQPGGSLRLSCRAS

SEQ ID NO: 180 - protein, 25 aa, synthetic construct
  REGION 1..25: note = FR1
EVQLVESGGGLVRPGGSLRLSCAAS

SEQ ID NO: 181 - protein, 25 aa, synthetic construct
  REGION 1..25: note = FR1
EVQLVESGGGLVQPGGSLRLSCVAS

SEQ ID NO: 182 - protein, 25 aa, synthetic construct
  REGION 1..25: note = FR1
EVQLVESGGGSVQPGGSLRLSCAAS

SEQ ID NO: 183 - protein, 25 aa, synthetic construct
  REGION 1..25: note = FR1
EVQLVESGGGLVQPGGSLRPSCAAS

SEQ ID NO: 184 - protein, 25 aa, synthetic construct
  REGION 1..25: note = FR1
EVQLVESGGGLVQPGGSLRLSCITS

SEQ ID NO: 185 - protein, 25 aa, synthetic construct
  REGION 1..25: note = FR1
EVQLVESGGGLVHPGGSLRLSCAAS

SEQ ID NO: 186 - protein, 25 aa, synthetic construct
  REGION 1..25: note = FR1
EVQLVESGGGLVQPGGSARLSCVAS

SEQ ID NO: 187 - protein, 25 aa, synthetic construct
  REGION 1..25: note = FR1
EVQLVESGGGLVQAGGSLTLSCAAS

SEQ ID NO: 188 - protein, 25 aa, synthetic construct
  REGION 1..25: note = FR1
EVQLVESGGDLVQPGGSLRLSCAAS

SEQ ID NO: 189 - protein, 25 aa, synthetic construct
  REGION 1..25: note = FR1
EVQLVESGGGLVQPEGSLRLSCAAS

SEQ ID NO: 190 - protein, 25 aa, synthetic construct
  REGION 1..25: note = FR1
EVQLVESGGGLVQPGGSLKLPCAAS

SEQ ID NO: 191 - protein, 25 aa, synthetic construct
  REGION 1..25: note = FR1
EVQLVESGGGLVQPGGSLGLSCAAS

SEQ ID NO: 192 - protein, 25 aa, synthetic construct
  REGION 1..25: note = FR1
EVQLVESGGGLAQPGGSLRLSCAAS

SEQ ID NO: 193 - protein, 25 aa, synthetic construct
  REGION 1..25: note = FR1
EVQLVESGGGWVQPGGSLRLSCAAS

SEQ ID NO: 194 - protein, 25 aa, synthetic construct
  REGION 1..25: note = FR1
EVQLVESGGGSVQPGGSLRPSCAAS

SEQ ID NO: 195 - protein, 25 aa, synthetic construct
  REGION 1..25: note = FR1
EVQLVESGGGLVQPGESLRLSCAAS

SEQ ID NO: 196 - protein, 26 aa, synthetic construct
  REGION 1..26: note = FR1
EVQLVEESGGGLVQPGGSLRLSCITS

SEQ ID NO: 197 - protein, 25 aa, synthetic construct
  REGION 1..25: note = FR1
EVQLVESGGGLVRPGGSLRLSCVAS

SEQ ID NO: 198 - protein, 25 aa, synthetic construct
  REGION 1..25: note = FR1
EVQLVESGGGMVQPGGSLRLSCAAS

SEQ ID NO: 199 - protein, 25 aa, synthetic construct
  REGION 1..25: note = FR1
EVQLVESGGGLVQPGGSLRLSCLTS

SEQ ID NO: 200 - protein, 25 aa, synthetic construct
  REGION 1..25: note = FR1
EVQLVESGGGLVQPGGSPRLSCVAS

SEQ ID NO: 201 - protein, 25 aa, synthetic construct
  REGION 1..25: note = FR1
EVQLVESGGGLVQPGGSLRPSCVAS

SEQ ID NO: 202 - protein, 25 aa, synthetic construct
  REGION 1..25: note = FR1
EVQLVESGGGWVQAGGSLRLSCAAS

SEQ ID NO: 203 - protein, 14 aa, synthetic construct
  REGION 1..14: note = FR2
WYRQAPGKERELVA

SEQ ID NO: 204 - protein, 14 aa, synthetic construct
  REGION 1..14: note = FR2
WYRQAPGKERGLVA

SEQ ID NO: 205 - protein, 14 aa, synthetic construct
  REGION 1..14: note = FR2
WYRQAPGKEREMVA

SEQ ID NO: 206 - protein, 14 aa, synthetic construct
  REGION 1..14: note = FR2
WYRQTPEKEREMVA

SEQ ID NO: 207 - protein, 14 aa, synthetic construct
  REGION 1..14: note = FR2
WYRQAPAKEREMVA

SEQ ID NO: 208 - protein, 14 aa, synthetic construct
  REGION 1..14: note = FR2
WYRQAPGKEREKVA

SEQ ID NO: 209 - protein, 14 aa, synthetic construct
  REGION 1..14: note = FR2
WYRQCPGKEREMVA

SEQ ID NO: 210 - protein, 14 aa, synthetic construct
  REGION 1..14: note = FR2
WYRQAPGKQRELVA

SEQ ID NO: 211 - protein, 14 aa, synthetic construct
  REGION 1..14: note = FR2
WHRQPPGKEREKVA

SEQ ID NO: 212 - protein, 14 aa, synthetic construct
  REGION 1..14: note = FR2
WYRQAPGKRRELVA

SEQ ID NO: 213 - protein, 14 aa, synthetic construct
  REGION 1..14: note = FR2
WHRQAPGKEREKVA

SEQ ID NO: 214 - protein, 14 aa, synthetic construct
  REGION 1..14: note = FR2
WYRQAPEKEREMVA

SEQ ID NO: 215 - protein, 14 aa, synthetic construct
  REGION 1..14: note = FR2
WYRQAPGKEREVVA

SEQ ID NO: 216 - protein, 14 aa, synthetic construct
  REGION 1..14: note = FR2
WYRQAPGKERGVVA

SEQ ID NO: 217 - protein, 14 aa, synthetic construct
  REGION 1..14: note = FR2
WYRQTPGKQRELVA

SEQ ID NO: 218 - protein, 14 aa, synthetic construct
  REGION 1..14: note = FR2
WYRQAPGKEREMVT

SEQ ID NO: 219 - protein, 14 aa, synthetic construct
  REGION 1..14: note = FR2
WYRQAPGHERELVA

SEQ ID NO: 220 - protein, 14 aa, synthetic construct
  REGION 1..14: note = FR2
WYRQAPGNQREVVA

SEQ ID NO: 221 - protein, 14 aa, synthetic construct
  REGION 1..14: note = FR2
WYRQAPGNQRGVVA

SEQ ID NO: 222 - protein, 14 aa, synthetic construct
  REGION 1..14: note = FR2
WYRQAPAKERGMVA

SEQ ID NO: 223 - protein, 14 aa, synthetic construct
  REGION 1..14: note = FR2
WYRQAPAKEHEMVA

SEQ ID NO: 224 - protein, 14 aa, synthetic construct
  REGION 1..14: note = FR2
WYRQAPAREREMVA

SEQ ID NO: 225 - protein, 14 aa, synthetic construct
  REGION 1..14: note = FR2
WYRQGPGKQRELVA

SEQ ID NO: 226 - protein, 14 aa, synthetic construct
  REGION 1..14: note = FR2
WYRQAPGKERGMVA

SEQ ID NO: 227 - protein, 14 aa, synthetic construct
  REGION 1..14: note = FR2
WYRQAPAKEREMIA

SEQ ID NO: 228 - protein, 14 aa, synthetic construct
  REGION 1..14: note = FR2
WYRQAPAKGREMVA

SEQ ID NO: 229 - protein, 14 aa, synthetic construct
  REGION 1..14: note = FR2
WYRQVPAKEREMVA

SEQ ID NO: 230 - protein, 14 aa, synthetic construct
  REGION 1..14: note = FR2
WYRQCPGKERDMVA

SEQ ID NO: 231 - protein, 14 aa, synthetic construct
  REGION 1..14: note = FR2
WQRQAPGKEREKVA

SEQ ID NO: 232 - protein, 14 aa, synthetic construct
  REGION 1..14: note = FR2
WYCQAPGKEREMVA

SEQ ID NO: 233 - protein, 14 aa, synthetic construct
  REGION 1..14: note = FR2
WYRQAPGKERDMVA

SEQ ID NO: 234 - protein, 14 aa, synthetic construct
  REGION 1..14: note = FR2
WHRQAPAKEREMVA

SEQ ID NO: 235 - protein, 39 aa, synthetic construct
  REGION 1..39: note = FR3
YADSAKGRFTISRDEAKNMVYLQMNSLKPEDTAVHFCRA

SEQ ID NO: 236 - protein, 39 aa, synthetic construct
  REGION 1..39: note = FR3
YADYAKGRFTISRDEARNMVYLQMNSLKPEDTAVYFCRA

SEQ ID NO: 237 - protein, 39 aa, synthetic construct
  REGION 1..39: note = FR3
YADSAKGRFTISRDEAKNMVYLQMNSLKPEDTAVYFCRA

SEQ ID NO: 238 - protein, 39 aa, synthetic construct
  REGION 1..39: note = FR3
YSHFAKGRFTISRDEAKNMVYLQMNSLRPEDTAVYFCRA

SEQ ID NO: 239 - protein, 39 aa, synthetic construct
  REGION 1..39: note = FR3
YADSAKGRFTISRDEAKNMVYLQMTSLKPEDTAVYVCRA

SEQ ID NO: 240 - protein, 39 aa, synthetic construct
  REGION 1..39: note = FR3
YAESAKGRFTISRDEAKNMVYLQMNSLKPEDTAVYFCRA

SEQ ID NO: 241 - protein, 39 aa, synthetic construct
  REGION 1..39: note = FR3
YADSAKGRFTISRDEAKNMVYLQMNSLSPEDTAVYFCRA

SEQ ID NO: 242 - protein, 39 aa, synthetic construct
  REGION 1..39: note = FR3
YAHFAKGRFTISRDEAKNMVYLQMNSLRPEDTAVYFCRA

SEQ ID NO: 243 - protein, 39 aa, synthetic construct
  REGION 1..39: note = FR3
YADSVKGRFTISEDSAKNTVYLQMNSLKAEDTAVYFCNA

SEQ ID NO: 244 - protein, 39 aa, synthetic construct
  REGION 1..39: note = FR3
YADSAKGRFTISRDEAKNMVYLQMTSLTPEDTAVYVCRA

SEQ ID NO: 245 - protein, 39 aa, synthetic construct
  REGION 1..39: note = FR3
YADSAKGRFTISRDEAKNMVYLQMNNLKPEDTAVYFCRA

SEQ ID NO: 246 - protein, 39 aa, synthetic construct
  REGION 1..39: note = FR3
YADSVKGRFTISEDSAKNTVYLQMNSLKPEDTAVYFCNA

SEQ ID NO: 247 - protein, 39 aa, synthetic construct
  REGION 1..39: note = FR3
YADSAKGRFTISRDEAKNMVHLQMNSLKPEDTAVYFCRA

SEQ ID NO: 248 - protein, 39 aa, synthetic construct
  REGION 1..39: note = FR3
YADSAKGRFTISRDEAKNMVFLQMNNLKPEDTAVYFCRA

SEQ ID NO: 249 - protein, 39 aa, synthetic construct
  REGION 1..39: note = FR3
YAGSAKGRFTISRDEAKNMVYLQMNSLKPEDTAVYFCRA

SEQ ID NO: 250 - protein, 39 aa, synthetic construct
  REGION 1..39: note = FR3
YADFAKGRFTISRDEAKNMVYLQMNSLKPEDTAVYFCRA

SEQ ID NO: 251 - protein, 39 aa, synthetic construct
  REGION 1..39: note = FR3
YADSAKGRFTISRDEAKNMVYLQMTSLKPEDTTVYVCRA

SEQ ID NO: 252 - protein, 39 aa, synthetic construct
  REGION 1..39: note = FR3
YAESAKGRFTISRDESKNMVYLQMNSLKPEDTAVYLCRA

SEQ ID NO: 253 - protein, 39 aa, synthetic construct
  REGION 1..39: note = FR3
YADSAKGRFAISRDEAKNMVYLQMNSLKPEDTAVYFCRA

SEQ ID NO: 254 - protein, 39 aa, synthetic construct
  REGION 1..39: note = FR3
YADFAQGRFTISRDEAKNMVYLQMNSLKPEDTAVYFCRA

SEQ ID NO: 255 - protein, 39 aa, synthetic construct
  REGION 1..39: note = FR3
YAEFAKGRFTISRDEPKNMVHLQMNSLKPEDTAVYLCRA

SEQ ID NO: 256 - protein, 39 aa, synthetic construct
  REGION 1..39: note = FR3
YADFAKGRLTISRDEAKNMVYLQMNSLKPEDTAVYFCRA

SEQ ID NO: 257 - protein, 39 aa, synthetic construct
  REGION 1..39: note = FR3
YADSAKGRFTISRDESKNMVYLQMNSLKPEDTAVYFCRA

SEQ ID NO: 258 - protein, 39 aa, synthetic construct
  REGION 1..39: note = FR3
YADFAKGRFTISRDGAKNMVYLQMNSLKPEDTAVYFCRA

SEQ ID NO: 259 - protein, 39 aa, synthetic construct
  REGION 1..39: note = FR3
YADSAKGRFTISRDEARNMVYLQMNSLKPEDTALYFCHA

SEQ ID NO: 260 - protein, 39 aa, synthetic construct
  REGION 1..39: note = FR3
YADSAKGRFTISRDEAKNMVYLQMNSLKPEDTAAYFCRA

SEQ ID NO: 261 - protein, 39 aa, synthetic construct
  REGION 1..39: note = FR3
YADSAKGRFTISRDESRNMVYLQMSSLKPEDTAVYFCHA

SEQ ID NO: 262 - protein, 39 aa, synthetic construct
  REGION 1..39: note = FR3
YADSAKGRFTISRDESRNMVYLQMGSLKPEDTAVYFCHA

SEQ ID NO: 263 - protein, 39 aa, synthetic construct
  REGION 1..39: note = FR3
YADSAKGRFTISRDEAENMVYLQMNSLKPEDTAVYFCRA

SEQ ID NO: 264 - protein, 39 aa, synthetic construct
  REGION 1..39: note = FR3
YADSAKGRFTISRDEATNMVYLQMTSLKPEDTAVYFCRA

SEQ ID NO: 265 - protein, 39 aa, synthetic construct
  REGION 1..39: note = FR3
YAGSAKGRFTISRDEAKNMVYLQLNNLKPEDTAVYFCRA

SEQ ID NO: 266 - protein, 39 aa, synthetic construct
  REGION 1..39: note = FR3
YADSAKGRFTISRDEAKNMVYLQLNNLKPEDTAVYFCRA

SEQ ID NO: 267 - protein, 39 aa, synthetic construct
  REGION 1..39: note = FR3
YAEFAKGRFTISRDEPKNMVYLQMNSLKPEDTAVYLCRA

SEQ ID NO: 268 - protein, 39 aa, synthetic construct
  REGION 1..39: note = FR3
YAHSAKGRFTISRDEAKNMVYLQMTSLKPEDTAVYVCRA

SEQ ID NO: 269 - protein, 39 aa, synthetic construct
  REGION 1..39: note = FR3
YADFAKGRFTISRDEVKNMVYLQMNSLKPEDTAVYFCRA

SEQ ID NO: 270 - protein, 39 aa, synthetic construct
  REGION 1..39: note = FR3
YADFAKGRFTISRDEAKNMVYLQMNSLRPEDTAVYFCRA

SEQ ID NO: 271 - protein, 39 aa, synthetic construct
  REGION 1..39: note = FR3
YSYFAKGRFTISRDEAKNMVYLQMNSLRPEDTAVYFCRA

SEQ ID NO: 272 - protein, 39 aa, synthetic construct
  REGION 1..39: note = FR3
YADSAKGRFTISRDEAKNVVYLQMNSLKPEDTAVYFCRA

SEQ ID NO: 273 - protein, 39 aa, synthetic construct
  REGION 1..39: note = FR3
YEDSAKGRFTISRDEAKNMVYLQMTGLKPEDTAVYVCRA

SEQ ID NO: 274 - protein, 39 aa, synthetic construct
  REGION 1..39: note = FR3
YADSVKGRFTISEDSAKNTVYLQMSSLKPEDTAVYFCNA

SEQ ID NO: 275 - protein, 39 aa, synthetic construct
  REGION 1..39: note = FR3
YSHFAKGRFTISRDEAKNMVYLQMNGLRPEDTAVYFCRA

SEQ ID NO: 276 - protein, 39 aa, synthetic construct
  REGION 1..39: note = FR3
YADSAKGRFTISRDEAKNMVYLQMNSLKPEDTAVYLCRA

SEQ ID NO: 277 - protein, 39 aa, synthetic construct
  REGION 1..39: note = FR3
YAEFAKGRFTISRDEPKNMVYLQMNSLKPVDTAVYLCRA

SEQ ID NO: 278 - protein, 39 aa, synthetic construct
  REGION 1..39: note = FR3
YSHFAKGRFTISRDEAKNMVYLQMNNLRPEDTAVYFCRA

SEQ ID NO: 279 - protein, 39 aa, synthetic construct
  REGION 1..39: note = FR3
YADSVKGRFTISEDSAKDTVYLQMNSLKPEDTAVYFCNA

SEQ ID NO: 280 - protein, 39 aa, synthetic construct
  REGION 1..39: note = FR3
YADSAKGRFTISRDEAKNMVYLQMNSLKPEDAAVYFCRA

SEQ ID NO: 281 - protein, 39 aa, synthetic construct
  REGION 1..39: note = FR3
YAESAKGRFTISRDESKNMVYLQMNSLKPEDAAVYLCRA

SEQ ID NO: 282 - protein, 39 aa, synthetic construct
  REGION 1..39: note = FR3
YADSAKGRFTISRDESRNMVYLQMSSLKPENTAVYFCHA

SEQ ID NO: 283 - protein, 39 aa, synthetic construct
  REGION 1..39: note = FR3
YADSAKGRFTISRDEAKNMVYLQMDSLKPEDTAVYFCRA

SEQ ID NO: 284 - protein, 39 aa, synthetic construct
  REGION 1..39: note = FR3
YADSAKGRFTISRDEAKNMVYLQMNSLKPGDTAVYFCRA

SEQ ID NO: 285 - protein, 11 aa, synthetic construct
  REGION 1..11: note = FR4
WGQGTQVTVSS

SEQ ID NO: 286 - protein, 11 aa, synthetic construct
  REGION 1..11: note = FR4
WGQGTLVTVSS

SEQ ID NO: 287 - protein, 11 aa, synthetic construct
  REGION 1..11: note = FR4
WGRGTQVTVSS

SEQ ID NO: 288 - protein, 11 aa, synthetic construct
  REGION 1..11: note = FR4
WGHGTLVTVSS

SEQ ID NO: 289 - protein, 11 aa, synthetic construct
  REGION 1..11: note = FR4
WGRGTLVTVSS

SEQ ID NO: 290 - protein, 11 aa, synthetic construct
  REGION 1..11: note = FR4
WDQGTQVTVSS

SEQ ID NO: 291 - protein, 327 aa, synthetic construct
  REGION 1..327: note = Nanobody sequence
EVQLVESGGGLVQGGGSLSLSCAASGRTFSSYAMAWFRQPPGKEREFVASISWSGENTNYRNSVKGRFTISRDNAKNTVYLQMNSLKPEDTAVYYCAAKIAKTYPDNWYWTKSNNYNYWGQGTLVTVSSGGGGSGGGGSGGGGSGGGGSGGGGSGGGGSGGGGSEVQLVESGGGLVQGGGSLSLSCAASGRTFSSYAMAWFRQPPGKEREFVASISWSGENTNYRNSVKGRFTISRDNAKNTVYLQMNSLKPEDTAVYYCAAKIAKTYPDNWYWTKSNNYNYWGQGTLVTVSSGAADYKDHDGDYKDHDIDYKDDDDKGAAHHHHHH

SEQ ID NO: 292 - protein, 276 aa, synthetic construct
  REGION 1..276: note = Nanobody sequence
EVQLVESGGGLVQPGGSLRLSCTFSGGTFSSYTMGWFRQAPGKEREFVAEVRWGGVTTYSNSLKDRFSISEDSVKNAVYLQMNSLKPEDTAVYYCAAVRQMYMTVVPDYWGQGTLVTVSSGGGGSEVQLVESGGGLVQPGGSLRLSCAASGSVHKINFLGWYRQAPGKERGLVATITIGDTTDYADYAKGRFTISRDEARNMVYLQMNSLKPEDTAVYFCRAGSRLYPYNYWGQGTLVTVSSGAADYKDHDGDYKDHDIDYKDDDDKGAAHHHHHH

SEQ ID NO: 293 - protein, 289 aa, synthetic construct
  REGION 1..289: note = Nanobody sequence
EVQLQASGGGSVQAGGSLRLSCAASGYTIGPYCMGWFRQAPGKEREGVAAINMGGGITYYADSVKGRFTISQDNAKNTVYLLMNSLEPEDTAIYYCAADSTIYASYYECGHGLSTGGYGYDSWGQGTQVTVSSGGGGSEVQLVESGGGLVQPGGSLRLSCAASGSVHKINFLGWYRQAPGKERGLVATITIGDTTDYADYAKGRFTISRDEARNMVYLQMNSLKPEDTAVYFCRAGSRLYPYNYWGQGTLVTVSSGAADYKDHDGDYKDHDIDYKDDDDKGAAHHHHHH

SEQ ID NO: 294 - protein, 292 aa, synthetic construct
  REGION 1..292: note = Nanobody sequence
EVQLVESGGGLVQPGGSLRLSCTFSGGTFSSYTMGWFRQAPGKEREFVAEVRWGGVTTYSNSLKDRFSISEDSVKNAVYLQMNSLKPEDTAVYYCAAVRQMYMTVVPDYWGQGTLVTVSSGGGGSDVQLQASGGGSVQAGGSLRLSCAASGYTIGPYCMGWFRQAPGKEREGVAAINMGGGITYYADSVKGRFTISQDNAKNTVYLLMNSLEPEDTAIYYCAADSTIYASYYECGHGLSTGGYGYDSWGQGTQVTVSSGAADYKDHDGDYKDHDIDYKDDDDKGAAHHHHHH

SEQ ID NO: 295 - protein, 276 aa, synthetic construct
  REGION 1..276: note = Nanobody sequence
EVQLVESGGGLVQPGGSLRLSCAASGSVHKINFLGWYRQAPGKERGLVATITIGDTTDYADYAKGRFTISRDEARNMVYLQMNSLKPEDTAVYFCRAGSRLYPYNYWGQGTLVTVSSGGGGSEVQLVESGGGLVQPGGSLRLSCTFSGGTFSSYTMGWFRQAPGKEREFVAEVRWGGVTTYSNSLKDRFSISEDSVKNAVYLQMNSLKPEDTAVYYCAAVRQMYMTVVPDYWGQGTLVTVSSGAADYKDHDGDYKDHDIDYKDDDDKGAAHHHHHH

SEQ ID NO: 296 - protein, 280 aa, synthetic construct
  REGION 1..280: note = Nanobody sequence
EVQLVESGGGLVQPGGSLRLSCTFSGGTFSSYTMGWFRQAPGKEREFVAEVRWGGVTTYSNSLKDRFSISEDSVKNAVYLQMNSLKPEDTAVYYCAAVRQMYMTVVPDYWGQGTLVTVSSGGGGSGGGSEVQLVESGGGLVQPGGSLRLSCAASGSVHKINFLGWYRQAPGKERGLVATITIGDTTDYADYAKGRFTISRDEARNMVYLQMNSLKPEDTAVYFCRAGSRLYPYNYWGQGTLVTVSSGAADYKDHDGDYKDHDIDYKDDDDKGAAHHHHHH

SEQ ID NO: 297 - protein, 293 aa, synthetic construct
  REGION 1..293: note = Nanobody sequence
EVQLQASGGGSVQAGGSLRLSCAASGYTIGPYCMGWFRQAPGKEREGVAAINMGGGITYYADSVKGRFTISQDNAKNTVYLLMNSLEPEDTAIYYCAADSTIYASYYECGHGLSTGGYGYDSWGQGTQVTVSSGGGGSGGGSEVQLVESGGGLVQPGGSLRLSCAASGSVHKINFLGWYRQAPGKERGLVATITIGDTTDYADYAKGRFTISRDEARNMVYLQMNSLKPEDTAVYFCRAGSRLYPYNYWGQGTLVTVSSGAADYKDHDGDYKDHDIDYKDDDDKGAAHHHHHH

SEQ ID NO: 298 - protein, 296 aa, synthetic construct
  REGION 1..296: note = Nanobody sequence
EVQLVESGGGLVQPGGSLRLSCTFSGGTFSSYTMGWFRQAPGKEREFVAEVRWGGVTTYSNSLKDRFSISEDSVKNAVYLQMNSLKPEDTAVYYCAAVRQMYMTVVPDYWGQGTLVTVSSGGGGSGGGSDVQLQASGGGSVQAGGSLRLSCAASGYTIGPYCMGWFRQAPGKEREGVAAINMGGGITYYADSVKGRFTISQDNAKNTVYLLMNSLEPEDTAIYYCAADSTIYASYYECGHGLSTGGYGYDSWGQGTQVTVSSGAADYKDHDGDYKDHDIDYKDDDDKGAAHHHHHH

SEQ ID NO: 299 - protein, 280 aa, synthetic construct
  REGION 1..280: note = Nanobody sequence
EVQLVESGGGLVQPGGSLRLSCAASGSVHKINFLGWYRQAPGKERGLVATITIGDTTDYADYAKGRFTISRDEARNMVYLQMNSLKPEDTAVYFCRAGSRLYPYNYWGQGTLVTVSSGGGGSGGGSEVQLVESGGGLVQPGGSLRLSCTFSGGTFSSYTMGWFRQAPGKEREFVAEVRWGGVTTYSNSLKDRFSISEDSVKNAVYLQMNSLKPEDTAVYYCAAVRQMYMTVVPDYWGQGTLVTVSSGAADYKDHDGDYKDHDIDYKDDDDKGAAHHHHHH

SEQ ID NO: 300 - protein, 306 aa, synthetic construct
  REGION 1..306: note = Nanobody sequence
EVQLVESGGGLVQPGGSLRLSCTFSGGTFSSYTMGWFRQAPGKEREFVAEVRWGGVTTYSNSLKDRFSISEDSVKNAVYLQMNSLKPEDTAVYYCAAVRQMYMTVVPDYWGQGTLVTVSSGGGGSGGGGSGGGGSGGGGSGGGGSGGGGSGGGGSEVQLVESGGGLVQPGGSLRLSCAASGSVHKINFLGWYRQAPGKERGLVATITIGDTTDYADYAKGRFTISRDEARNMVYLQMNSLKPEDTAVYFCRAGSRLYPYNYWGQGTLVTVSSGAADYKDHDGDYKDHDIDYKDDDDKGAAHHHHHH

SEQ ID NO: 301 - protein, 319 aa, synthetic construct
  REGION 1..319: note = Nanobody sequence
EVQLQASGGGSVQAGGSLRLSCAASGYTIGPYCMGWFRQAPGKEREGVAAINMGGGITYYADSVKGRFTISQDNAKNTVYLLMNSLEPEDTAIYYCAADSTIYASYYECGHGLSTGGYGYDSWGQGTQVTVSSGGGGSGGGGSGGGGSGGGGSGGGGSGGGGSGGGGSEVQLVESGGGLVQPGGSLRLSCAASGSVHKINFLGWYRQAPGKERGLVATITIGDTTDYADYAKGRFTISRDEARNMVYLQMNSLKPEDTAVYFCRAGSRLYPYNYWGQGTLVTVSSGAADYKDHDGDYKDHDIDYKDDDDKGAAHHHHHH

SEQ ID NO: 302 - protein, 322 aa, synthetic construct
  REGION 1..322: note = Nanobody sequence
EVQLVESGGGLVQPGGSLRLSCTFSGGTFSSYTMGWFRQAPGKEREFVAEVRWGGVTTYSNSLKDRFSISEDSVKNAVYLQMNSLKPEDTAVYYCAAVRQMYMTVVPDYWGQGTLVTVSSGGGGSGGGGSGGGGSGGGGSGGGGSGGGGSGGGGSDVQLQASGGGSVQAGGSLRLSCAASGYTIGPYCMGWFRQAPGKEREGVAAINMGGGITYYADSVKGRFTISQDNAKNTVYLLMNSLEPEDTAIYYCAADSTIYASYYECGHGLSTGGYGYDSWGQGTQVTVSSGAADYKDHDGDYKDHDIDYKDDDDKGAAHHHHHH

SEQ ID NO: 303 - protein, 306 aa, synthetic construct
  REGION 1..306: note = Nanobody sequence
EVQLVESGGGLVQPGGSLRLSCAASGSVHKINFLGWYRQAPGKERGLVATITIGDTTDYADYAKGRFTISRDEARNMVYLQMNSLKPEDTAVYFCRAGSRLYPYNYWGQGTLVTVSSGGGGSGGGGSGGGGSGGGGSGGGGSGGGGSGGGGSEVQLVESGGGLVQPGGSLRLSCTFSGGTFSSYTMGWFRQAPGKEREFVAEVRWGGVTTYSNSLKDRFSISEDSVKNAVYLQMNSLKPEDTAVYYCAAVRQMYMTVVPDYWGQGTLVTVSSGAADYKDHDGDYKDHDIDYKDDDDKGAAHHHHHH

SEQ ID NO: 304 - protein, 322 aa, synthetic construct
  REGION 1..322: note = Nanobody sequence
EVQLQASGGGSVQAGGSLRLSCAASGYTIGPYCMGWFRQAPGKEREGVAAINMGGGITYYADSVKGRFTISQDNAKNTVYLLMNSLEPEDTAIYYCAADSTIYASYYECGHGLSTGGYGYDSWGQGTQVTVSSGGGGSGGGGSGGGGSGGGGSGGGGSGGGGSGGGGSEVQLVESGGGLVQPGGSLRLSCTFSGGTFSSYTMGWFRQAPGKEREFVAEVRWGGVTTYSNSLKDRFSISEDSVKNAVYLQMNSLKPEDTAVYYCAAVRQMYMTVVPDYWGQGTLVTVSSGAADYKDHDGDYKDHDIDYKDDDDKGAAHHHHHH

SEQ ID NO: 305 - protein, 319 aa, synthetic construct
  REGION 1..319: note = Nanobody sequence
EVQLVESGGGLVQPGGSLRLSCAASGSVHKINFLGWYRQAPGKERGLVATITIGDTTDYADYAKGRFTISRDEARNMVYLQMNSLKPEDTAVYFCRAGSRLYPYNYWGQGTLVTVSSGGGGSGGGGSGGGGSGGGGSGGGGSGGGGSGGGGSDVQLQASGGGSVQAGGSLRLSCAASGYTIGPYCMGWFRQAPGKEREGVAAINMGGGITYYADSVKGRFTISQDNAKNTVYLLMNSLEPEDTAIYYCAADSTIYASYYECGHGLSTGGYGYDSWGQGTQVTVSSGAADYKDHDGDYKDHDIDYKDDDDKGAAHHHHHH

SEQ ID NO: 306 - protein, 306 aa, synthetic construct
  REGION 1..306: note = Nanobody sequence
EVQLVESGGGLVQPGGSLRLSCAASGDVYKINFLGWHRQAPGKEREKVAHITIGDATDYADSAKGRFTISRDEAKNMVYLQMNSLKPEDTAVYFCRAGSRIYPYDYWGQGTLVTVSSGGGGSGGGGSGGGGSGGGGSGGGGSGGGGSGGGGSEVQLVESGGGLVQPGGSLRLSCTFSGGTFSSYTMGWFRQAPGKEREFVAEVRWGGVTTYSNSLKDRFSISEDSVKNAVYLQMNSLKPEDTAVYYCAAVRQMYMTVVPDYWGQGTLVTVSSGAADYKDHDGDYKDHDIDYKDDDDKGAAHHHHHH

SEQ ID NO: 307 - protein, 306 aa, synthetic construct
  REGION 1..306: note = Nanobody sequence
EVQLVESGGGLVQPGGSLKLSCAASGAVHKINFLGWYRQTPEKEREMVATITIGDEVDYADSAKGRFTISRDEAKNMVYLQMTSLKPEDTAVYVCRAGSRLYPYNYWGQGTLVTVSSGGGGSGGGGSGGGGSGGGGSGGGGSGGGGSGGGGSEVQLVESGGGLVQPGGSLRLSCTFSGGTFSSYTMGWFRQAPGKEREFVAEVRWGGVTTYSNSLKDRFSISEDSVKNAVYLQMNSLKPEDTAVYYCAAVRQMYMTVVPDYWGQGTLVTVSSGAADYKDHDGDYKDHDIDYKDDDDKGAAHHHHHH

SEQ ID NO: 308 - protein, 306 aa, synthetic construct
  REGION 1..306: note = Nanobody sequence
EVQLVESGGGLVQPGGSLRLSCITSGETFKINIWGWYRQAPGKQRELVASLTIGGATNYADSVKGRFTISEDSAKNTVYLQMNSLKPEDTAVYFCNAKSRLYPYDYWGQGTLVTVSSGGGGSGGGGSGGGGSGGGGSGGGGSGGGGSGGGGSEVQLVESGGGLVQPGGSLRLSCTFSGGTFSSYTMGWFRQAPGKEREFVAEVRWGGVTTYSNSLKDRFSISEDSVKNAVYLQMNSLKPEDTAVYYCAAVRQMYMTVVPDYWGQGTLVTVSSGAADYKDHDGDYKDHDIDYKDDDDKGAAHHHHHH

SEQ ID NO: 309 - protein, 306 aa, synthetic construct
  REGION 1..306: note = Nanobody sequence
EVQLVESGGGLVQPGGSLRLSCAASGSVHLLNFLGWYRQAPGKEREMVAHITIADATDYAHFAKGRFTISRDEAKNMVYLQMNSLRPEDTAVYFCRAGSRIYPYDYWGQGTLVTVSSGGGGSGGGGSGGGGSGGGGSGGGGSGGGGSGGGGSEVQLVESGGGLVQPGGSLRLSCTFSGGTFSSYTMGWFRQAPGKEREFVAEVRWGGVTTYSNSLKDRFSISEDSVKNAVYLQMNSLKPEDTAVYYCAAVRQMYMTVVPDYWGQGTLVTVSSGAADYKDHDGDYKDHDIDYKDDDDKGAAHHHHHH

SEQ ID NO: 310 - protein, 306 aa, synthetic construct
  REGION 1..306: note = Nanobody sequence
EVQLVESGGGLVQPGGSLRLSCITSGETFKINIWGWYRQAPGKQRELVASLTIGGATDYADSVKGRFTISEDSAKNTVYLQMNSLKAEDTAVYFCNAKSRLYPYDYWGQGTLVTVSSGGGGSGGGGSGGGGSGGGGSGGGGSGGGGSGGGGSEVQLVESGGGLVQPGGSLRLSCTFSGGTFSSYTMGWFRQAPGKEREFVAEVRWGGVTTYSNSLKDRFSISEDSVKNAVYLQMNSLKPEDTAVYYCAAVRQMYMTVVPDYWGQGTLVTVSSGAADYKDHDGDYKDHDIDYKDDDDKGAAHHHHHH

SEQ ID NO: 311 - protein, 306 aa, synthetic construct
  REGION 1..306: note = Nanobody sequence
EVQLVESGGGLVQPGGSLRLSCAASGEVYKINFLGWYRQAPGKEREKVAHITIADAADYADFAKGRFTISRDEAKNMVYLQMNSLRPEDTAVYFCRAGSRIWPYDYWGQGTLVTVSSGGGGSGGGGSGGGGSGGGGSGGGGSGGGGSGGGGSEVQLVESGGGLVQPGGSLRLSCTFSGGTFSSYTMGWFRQAPGKEREFVAEVRWGGVTTYSNSLKDRFSISEDSVKNAVYLQMNSLKPEDTAVYYCAAVRQMYMTVVPDYWGQGTLVTVSSGAADYKDHDGDYKDHDIDYKDDDDKGAAHHHHHH

SEQ ID NO: 312 - protein, 306 aa, synthetic construct
  REGION 1..306: note = Nanobody sequence
EVQLVESGGGLVQPGGSLRLSCVASGDVHKINFLGWYRQAPGKEREKVAHISIGDQTDYADSAKGRFTISRDESKNMVYLQMNSLKPEDTAVYFCRAFSRIYPYDYWGQGTLVTVSSGGGGSGGGGSGGGGSGGGGSGGGGSGGGGSGGGGSEVQLVESGGGLVQPGGSLRLSCTFSGGTFSSYTMGWFRQAPGKEREFVAEVRWGGVTTYSNSLKDRFSISEDSVKNAVYLQMNSLKPEDTAVYYCAAVRQMYMTVVPDYWGQGTLVTVSSGAADYKDHDGDYKDHDIDYKDDDDKGAAHHHHHH

SEQ ID NO: 313 - protein, 306 aa, synthetic construct
  REGION 1..306: note = Nanobody sequence
EVQLVESGGGLVQPGGSLRLSCAASGEIGRINFYRWYRQAPGNQREVVATITIADKTDYADSAKGRFTISRDESRNMVYLQMSSLKPEDTAVYFCHAGSRLYPYDYWGQGTLVTVSSGGGGSGGGGSGGGGSGGGGSGGGGSGGGGSGGGGSEVQLVESGGGLVQPGGSLRLSCTFSGGTFSSYTMGWFRQAPGKEREFVAEVRWGGVTTYSNSLKDRFSISEDSVKNAVYLQMNSLKPEDTAVYYCAAVRQMYMTVVPDYWGQGTLVTVSSGAADYKDHDGDYKDHDIDYKDDDDKGAAHHHHHH

SEQ ID NO: 314 - protein, 306 aa, synthetic construct
  REGION 1..306: note = Nanobody sequence
EVQLVESGGGLVQPGGSLRLSCVASGDVHKINFLGWYRQAPGKEREKVAHITIGDQADYADSAKGRFTISRDEAKNMVYLQMNSLKPEDTAVYFCRAGSRIYPYDYWGQGTLVTVSSGGGGSGGGGSGGGGSGGGGSGGGGSGGGGSGGGGSEVQLVESGGGLVQPGGSLRLSCTFSGGTFSSYTMGWFRQAPGKEREFVAEVRWGGVTTYSNSLKDRFSISEDSVKNAVYLQMNSLKPEDTAVYYCAAVRQMYMTVVPDYWGQGTLVTVSSGAADYKDHDGDYKDHDIDYKDDDDKGAAHHHHHH

SEQ ID NO: 315 - protein, 306 aa, synthetic construct
  REGION 1..306: note = Nanobody sequence
EVQLVESGGGLVQPGGSLRLSCAASGDVHKINILGWYRQAPAKEREMVAHITIGDATDYADSAKGRFTISRDEAKNMVYLQMNSLKPEDTAVYFCRAYSRIYPYNYWGQGTLVTVSSGGGGSGGGGSGGGGSGGGGSGGGGSGGGGSGGGGSEVQLVESGGGLVQPGGSLRLSCTFSGGTFSSYTMGWFRQAPGKEREFVAEVRWGGVTTYSNSLKDRFSISEDSVKNAVYLQMNSLKPEDTAVYYCAAVRQMYMTVVPDYWGQGTLVTVSSGAADYKDHDGDYKDHDIDYKDDDDKGAAHHHHHH

SEQ ID NO: 316 - protein, 306 aa, synthetic construct
  REGION 1..306: note = Nanobody sequence
EVQLVESGGGLVQPGGSLRLSCAASGSVHKINFLGWYRQAPGKERELVATITIGDTTDYADSAKGRFTISRDEAKNMVYLQMNSLKPEDTAVYFCRAGSRLYPYNYWGQGTLVTVSSGGGGSGGGGSGGGGSGGGGSGGGGSGGGGSGGGGSEVQLVESGGGLVQPGGSLRLSCTFSGGTFSSYTMGWFRQAPGKEREFVAEVRWGGVTTYSNSLKDRFSISEDSVKNAVYLQMNSLKPEDTAVYYCAAVRQMYMTVVPDYWGQGTLVTVSSGAADYKDHDGDYKDHDIDYKDDDDKGAAHHHHHH

SEQ ID NO: 317 - protein, 306 aa, synthetic construct; identical to SEQ ID NO: 303
  REGION 1..306: note = Nanobody sequence

SEQ ID NO: 318 - protein, 306 aa, synthetic construct
  REGION 1..306: note = Nanobody sequence
EVQLVESGGGLVQPGGSLRLSCAASGDVHKINILGWYRQAPAKEREMVAHITIGDATDYADSAKGRFTISRDEAKNMVYLQMNSLKPEDTAVYLCRAYSRIYPYNYWGQGTLVTVSSGGGGSGGGGSGGGGSGGGGSGGGGSGGGGSGGGGSEVQLVESGGGLVQPGGSLRLSCTFSGGTFSSYTMGWFRQAPGKEREFVAEVRWGGVTTYSNSLKDRFSISEDSVKNAVYLQMNSLKPEDTAVYYCAAVRQMYMTVVPDYWGQGTLVTVSSGAADYKDHDGDYKDHDIDYKDDDDKGAAHHHHHH

SEQ ID NO: 319 - protein, 306 aa, synthetic construct
  REGION 1..306: note = Nanobody sequence
EVQLVESGGGLVQPGGSLRLSCTFSGGTFSSYTMGWFRQAPGKEREFVAEVRWGGVTTYSNSLKDRFSISEDSVKNAVYLQMNSLKPEDTAVYYCAAVRQMYMTVVPDYWGQGTLVTVSSGGGGSGGGGSGGGGSGGGGSGGGGSGGGGSGGGGSEVQLVESGGGLVQPGGSLRLSCVASGDVHKINFLGWYRQAPGKEREKVAHISIGDQTDYADSAKGRFTISRDESKNMVYLQMNSLKPEDTAVYFCRAFSRIYPYDYWGQGTLVTVSSGAADYKDHDGDYKDHDIDYKDDDDKGAAHHHHHH

SEQ ID NO: 320 - protein, 306 aa, synthetic construct
  REGION 1..306: note = Nanobody sequence
EVQLVESGGGLVQPGGSLRLSCTFSGGTFSSYTMGWFRQAPGKEREFVAEVRWGGVTTYSNSLKDRFSISEDSVKNAVYLQMNSLKPEDTAVYYCAAVRQMYMTVVPDYWGQGTLVTVSSGGGGSGGGGSGGGGSGGGGSGGGGSGGGGSGGGGSEVQLVESGGGLVQPGGSLRLSCAASGEIGRINFYRWYRQAPGNQREVVATITIADKTDYADSAKGRFTISRDESRNMVYLQMSSLKPEDTAVYFCHAGSRLYPYDYWGQGTLVTVSSGAADYKDHDGDYKDHDIDYKDDDDKGAAHHHHHH

SEQ ID NO: 321 - protein, 306 aa, synthetic construct
  REGION 1..306: note = Nanobody sequence
EVQLVESGGGLVQPGGSLRLSCTFSGGTFSSYTMGWFRQAPGKEREFVAEVRWGGVTTYSNSLKDRFSISEDSVKNAVYLQMNSLKPEDTAVYYCAAVRQMYMTVVPDYWGQGTLVTVSSGGGGSGGGGSGGGGSGGGGSGGGGSGGGGSGGGGSEVQLVESGGGLVQPGGSLRLSCVASGDVHKINFLGWYRQAPGKEREKVAHITIGDQADYADSAKGRFTISRDEAKNMVYLQMNSLKPEDTAVYFCRAGSRIYPYDYWGQGTLVTVSSGAADYKDHDGDYKDHDIDYKDDDDKGAAHHHHHH

SEQ ID NO: 322 - protein, 306 aa, synthetic construct
  REGION 1..306: note = Nanobody sequence
EVQLVESGGGLVQPGGSLRLSCTFSGGTFSSYTMGWFRQAPGKEREFVAEVRWGGVTTYSNSLKDRFSISEDSVKNAVYLQMNSLKPEDTAVYYCAAVRQMYMTVVPDYWGQGTLVTVSSGGGGSGGGGSGGGGSGGGGSGGGGSGGGGSGGGGSEVQLVESGGGLVQPGGSLRLSCAASGDVHKINILGWYRQAPAKEREMVAHITIGDATDYADSAKGRFTISRDEAKNMVYLQMNSLKPEDTAVYFCRAYSRIYPYNYWGQGTLVTVSSGAADYKDHDGDYKDHDIDYKDDDDKGAAHHHHHH

SEQ ID NO: 323 - protein, 306 aa, synthetic construct
  REGION 1..306: note = Nanobody sequence
EVQLVESGGGLVQPGGSLRLSCTFSGGTFSSYTMGWFRQAPGKEREFVAEVRWGGVTTYSNSLKDRFSISEDSVKNAVYLQMNSLKPEDTAVYYCAAVRQMYMTVVPDYWGQGTLVTVSSGGGGSGGGGSGGGGSGGGGSGGGGSGGGGSGGGGSEVQLVESGGGLVQPGGSLRLSCAASGSVHKINFLGWYRQAPGKERELVATITIGDTTDYADSAKGRFTISRDEAKNMVYLQMNSLKPEDTAVYFCRAGSRLYPYNYWGQGTLVTVSSGAADYKDHDGDYKDHDIDYKDDDDKGAAHHHHHH

SEQ ID NO: 324 - protein, 306 aa, synthetic construct; identical to SEQ ID NO: 300
  REGION 1..306: note = Nanobody sequence

SEQ ID NO: 325 - protein, 306 aa, synthetic construct
  REGION 1..306: note = Nanobody sequence
EVQLVESGGGLVQPGGSLRLSCTFSGGTFSSYTMGWFRQAPGKEREFVAEVRWGGVTTYSNSLKDRFSISEDSVKNAVYLQMNSLKPEDTAVYYCAAVRQMYMTVVPDYWGQGTLVTVSSGGGGSGGGGSGGGGSGGGGSGGGGSGGGGSGGGGSEVQLVESGGGLVQPGGSLRLSCAASGDVYKINFLGWHRQAPGKEREKVAHITIGDATDYADSAKGRFTISRDEAKNMVYLQMNSLKPEDTAVYFCRAGSRIYPYDYWGQGTLVTVSSGAADYKDHDGDYKDHDIDYKDDDDKGAAHHHHHH

SEQ ID NO: 326 - protein, 306 aa, synthetic construct
  REGION 1..306: note = Nanobody sequence
EVQLVESGGGLVQPGGSLRLSCTFSGGTFSSYTMGWFRQAPGKEREFVAEVRWGGVTTYSNSLKDRFSISEDSVKNAVYLQMNSLKPEDTAVYYCAAVRQMYMTVVPDYWGQGTLVTVSSGGGGSGGGGSGGGGSGGGGSGGGGSGGGGSGGGGSEVQLVESGGGLVQPGGSLRLSCAASGEVYKINFLGWYRQAPGKEREKVAHITIADAADYADFAKGRFTISRDEAKNMVYLQMNSLRPEDTAVYFCRAGSRIWPYDYWGQGTLVTVSSGAADYKDHDGDYKDHDIDYKDDDDKGAAHHHHHH

SEQ ID NO: 327 - protein, 306 aa, synthetic construct
  REGION 1..306: note = Nanobody sequence
EVQLVESGGGLVQPGGSLRLSCTFSGGTFSSYTMGWFRQAPGKEREFVAEVRWGGVTTYSNSLKDRFSISEDSVKNAVYLQMNSLKPEDTAVYYCAAVRQMYMTVVPDYWGQGTLVTVSSGGGGSGGGGSGGGGSGGGGSGGGGSGGGGSGGGGSEVQLVESGGDLVQPGGSLRLSCAASGDVHKINFLGWYRQAPGKEREMVAHITIADATDYAEFAKGRFTISRDEPKNMVYLQMNSLKPEDTAVYLCRAGSRIYPYNYWGQGTLVTVSSGAADYKDHDGDYKDHDIDYKDDDDKGAAHHHHHH

SEQ ID NO: 328 - protein, 306 aa, synthetic construct
  REGION 1..306: note = Nanobody sequence
EVQLVESGGGLVQPGGSLRLSCTFSGGTFSSYTMGWFRQAPGKEREFVAEVRWGGVTTYSNSLKDRFSISEDSVKNAVYLQMNSLKPEDTAVYYCAAVRQMYMTVVPDYWGQGTLVTVSSGGGGSGGGGSGGGGSGGGGSGGGGSGGGGSGGGGSEVQLVESGGGLVQPGGSLRLSCITSGETFKINIWGWYRQAPGKQRELVASLTIGGATNYADSVKGRFTISEDSAKNTVYLQMNSLKPEDTAVYFCNAKSRLYPYDYWGQGTLVTVSSGAADYKDHDGDYKDHDIDYKDDDDKGAAHHHHHH

SEQ ID NO: 329 - protein, 306 aa, synthetic construct
  REGION 1..306: note = Nanobody sequence
EVQLVESGGGLVQPGGSLRLSCTFSGGTFSSYTMGWFRQAPGKEREFVAEVRWGGVTTYSNSLKDRFSISEDSVKNAVYLQMNSLKPEDTAVYYCAAVRQMYMTVVPDYWGQGTLVTVSSGGGGSGGGGSGGGGSGGGGSGGGGSGGGGSGGGGSEVQLVESGGGLVQPGGSLRLSCAASGSVHLLNFLGWYRQAPGKEREMVAHITIADATDYAHFAKGRFTISRDEAKNMVYLQMNSLRPEDTAVYFCRAGSRIYPYDYWGQGTLVTVSSGAADYKDHDGDYKDHDIDYKDDDDKGAAHHHHHH

SEQ ID NO: 330 - protein, 306 aa, synthetic construct
  REGION 1..306: note = Nanobody sequence
EVQLVESGGGLVQPGGSLRLSCTFSGGTFSSYTMGWFRQAPGKEREFVAEVRWGGVTTYSNSLKDRFSISEDSVKNAVYLQMNSLKPEDTAVYYCAAVRQMYMTVVPDYWGQGTLVTVSSGGGGSGGGGSGGGGSGGGGSGGGGSGGGGSGGGGSEVQLVESGGGLVQPGGSLRLSCITSGETFKINIWGWYRQAPGKQRELVASLTIGGATDYADSVKGRFTISEDSAKNTVYLQMNSLKAEDTAVYFCNAKSRLYPYDYWGQGTLVTVSSGAADYKDHDGDYKDHDIDYKDDDDKGAAHHHHHH

SEQ ID NO: 331 - protein, 306 aa, synthetic construct
  REGION 1..306: note = Nanobody sequence
EVQLVESGGGLVQPGGSLRLSCAASGDVHKINILGWYRQAPAKEREMVAHITIGDATSYADSAKGRFTISRDEAKNMVYLQLNNLKPEDTAVYFCRAYSRIYPYNYWGQGTLVTVSSGGGGSGGGGSGGGGSGGGGSGGGGSGGGGSGGGGSEVQLVESGGGLVQPGGSLRLSCTFSGGTFSSYTMGWFRQAPGKEREFVAEVRWGGVTTYSNSLKDRFSISEDSVKNAVYLQMNSLKPEDTAVYYCAAVRQMYMTVVPDYWGQGTLVTVSSGAADYKDHDGDYKDHDIDYKDDDDKGAAHHHHHH

SEQ ID NO: 332 - protein, 306 aa, synthetic construct; identical to SEQ ID NO: 312
  REGION 1..306: note = Nanobody sequence

SEQ ID NO: 333 - protein, 306 aa, synthetic construct
  REGION 1..306: note = Nanobody sequence
EVQLVESGGGLVQPGGSLRLSCTFSGGTFSSYTMGWFRQAPGKEREFVAEVRWGGVTTYSNSLKDRFSISEDSVKNAVYLQMNSLKPEDTAVYYCAAVRQMYMTVVPDYWGQGTLVTVSSGGGGSGGGGSGGGGSGGGGSGGGGSGGGGSGGGGSEVQLVESGGGLVQPGGSLRLSCAASGDVHKINILGWYRQAPAKEREMVAHITIGDATSYADSAKGRFTISRDEAKNMVYLQLNNLKPEDTAVYFCRAYSRIYPYNYWGQGTLVTVSSGAADYKDHDGDYKDHDIDYKDDDDKGAAHHHHHH

SEQ ID NO: 334 - protein, 306 aa, synthetic construct; identical to SEQ ID NO: 319
  REGION 1..306: note = Nanobody sequence

SEQ ID NO: 335 - protein, 306 aa, synthetic construct
  REGION 1..306: note = Nanobody sequence
EVQLVESGGDLVQPGGSLRLSCAASGDVHKINFLGWYRQAPGKEREMVAHITIADATDYAEFAKGRFTISRDEPKNMVYLQMNSLKPEDTAVYLCRAGSRIYPYNYWGQGTLVTVSSGGGGSGGGGSGGGGSGGGGSGGGGSGGGGSGGGGSEVQLVESGGGLVQPGGSLRLSCTFSGGTFSSYTMGWFRQAPGKEREFVAEVRWGGVTTYSNSLKDRFSISEDSVKNAVYLQMNSLKPEDTAVYYCAAVRQMYMTVVPDYWGQGTLVTVSSGAADYKDHDGDYKDHDIDYKDDDDKGAAHHHHHH

SEQ ID NO: 336 - protein, 306 aa, synthetic construct
  REGION 1..306: note = Nanobody sequence
EVQLVESGGGLVQPGGSLRLSCTFSGGTFSSYTMGWFRQAPGKEREFVAEVRWGGVTTYSNSLKDRFSISEDSVKNAVYLQMNSLKPEDTAVYYCAAVRQMYMTVVPDYWGQGTLVTVSSGGGGSGGGGSGGGGSGGGGSGGGGSGGGGSGGGGSEVQLVESGGGLVQPGGSLRLSCAASGDVHKINILGWYRQAPAKEREMVAHITIGDATDYADSAKGRFTISRDEAKNMVYLQMNSLKPEDTAVYLCRAYSRIYPYNYWGQGTLVTVSSGAADYKDHDGDYKDHDIDYKDDDDKGAAHHHHHH

SEQ ID NO: 337 - protein, 306 aa, synthetic construct
  REGION 1..306: note = Nanobody sequence
EVQLVESGGGLVQPGGSLRLSCTFSGGTFSSYTMGWFRQAPGKEREFVAEVRWGGVTTYSNSLKDRFSISEDSVKNAVYLQMNSLKPEDTAVYYCAAVRQMYMTVVPDYWGQGTLVTVSSGGGGSGGGGSGGGGSGGGGSGGGGSGGGGSGGGGSEVQLVESGGGLVQPGGSLKLSCAASGAVHKINFLGWYRQTPEKEREMVATITIGDEVDYADSAKGRFTISRDEAKNMVYLQMTSLKPEDTAVYVCRAGSRLYPYNYWGQGTLVTVSSGAADYKDHDGDYKDHDIDYKDDDDKGAAHHHHHH

SEQ ID NO: 338 - protein, 273 aa, synthetic construct
  REGION 1..273: note = Nanobody sequence
DVQLVESGGGLVQPGGSLRLSCTFSGGTFSSYTMGWFRQAPGKEREFVAEVRWGGVTTYSNSLKDRFSISEDSVKNAVYLQMNSLKPEDTAVYYCAAVRQMYMTVVPDYWGQGTLVTVSSGGGGSGGGGSGGGGSGGGGSGGGGSGGGGSGGGGSEVQLVESGGGLVQPGGSLRLSCAASGDVHKINILGWYRQAPAKEREMVAHITIGDATDYADSAKGRFTISRDEAKNMVYLQMNSLKPEDTAVYFCRAYSRIYPYNYWGQGTLVTVSSA

SEQ ID NO: 339 - protein, 280 aa, synthetic construct
  REGION 1..280: note = Nanobody sequence
DVQLVESGGGLVQAGDSLRLSCAASGRTFSSYAMGWFRQAPGKEREFVAAISWSDGSTYYADSVKGRFTISRDNAKNTVYLQMNSLKPEDTAVYYCAADLTSTNPGSYIYIWAYDYWGQGTQVTVSSGGGGSGGGGSGGGGSGGGGSGGGGSGGGGSGGGGSEVQLVESGGGLVQPGGSLRLSCAASGDVHKINILGWYRQAPAKEREMVAHITIGDATDYADSAKGRFTISRDEAKNMVYLQMNSLKPEDTAVYFCRAYSRIYPYNYWGQGTLVTVSSA

SEQ ID NO: 340 - protein, 456 aa, synthetic construct
  REGION 1..456: note = Nanobody sequence
EVQLVESGGGLVQPGGSLRLSCTFSGGTFSSYTMGWFRQAPGKEREFVAEVRWGGVTTYSNSLKDRFSISEDSVKNAVYLQMNSLKPEDTAVYYCAAVRQMYMTVVPDYWGQGTLVTVSSGGGGSGGGGSGGGGSGGGGSGGGGSGGGGSGGGGSEVQLVESGGGLVQPGGSLRLSCVASGDVHKINFLGWYRQAPGKEREKVAHISIGDQTDYADSAKGRFTISRDESKNMVYLQMNSLKPEDTAVYFCRAFSRIYPYDYWGQGTLVTVSSGGGGSGGGGSGGGGSGGGGSGGGGSGGGGSGGGGSEVQLVESGGGLVQPGNSLRLSCAASGFTFSSFGMSWVRQAPGKGLEWVSSISGSGSDTLYADSVKGRFTISRDNAKTTLYLQMNSLRPEDTAVYYCTIGGSLSRSSQGTLVTVSSGAADYKDHDGDYKDHDIDYKDDDDKGAAHHHHHH

SEQ ID NO: 341 - protein, 456 aa, synthetic construct
  REGION 1..456: note = Nanobody sequence
EVQLVESGGGLVQPGGSLRLSCTFSGGTFSSYTMGWFRQAPGKEREFVAEVRWGGVTTYSNSLKDRFSISEDSVKNAVYLQMNSLKPEDTAVYYCAAVRQMYMTVVPDYWGQGTLVTVSSGGGGSGGGGSGGGGSGGGGSGGGGSGGGGSGGGGSEVQLVESGGGLVQPGGSLRLSCITSGETFKINIWGWYRQAPGKQRELVASLTIGGATNYADSVKGRFTISEDSAKNTVYLQMNSLKPEDTAVYFCNAKSRLYPYDYWGQGTLVTVSSGGGGSGGGGSGGGGSGGGGSGGGGSGGGGSGGGGSEVQLVESGGGLVQPGNSLRLSCAASGFTFSSFGMSWVRQAPGKGLEWVSSISGSGSDTLYADSVKGRFTISRDNAKTTLYLQMNSLRPEDTAVYYCTIGGSLSRSSQGTLVTVSSGAADYKDHDGDYKDHDIDYKDDDDKGAAHHHHHH

SEQ ID NO: 342 - protein, 304 aa, synthetic construct
  REGION 1..304: note = Nanobody sequence
EVQLVESGGGLVQAGGSLRLSCAASGITFSINTMGWYRQAPGKQRELVALISSIGDTYYADSVKGRFTISRDNAKNTVYLQMNSLKPEDTAVYYCKRFRTAAQGTDYWGQGTLVTVSSGGGGSGGGGSGGGGSGGGGSGGGGSGGGGSGGGGSEVQLVESGGGLVQPGGSLRLSCVASGDVHKINFLGWYRQAPGKEREKVAHISIGDQTDYADSAKGRFTISRDESKNMVYLQMNSLKPEDTAVYFCRAFSRIYPYDYWGQGTLVTVSSGAADYKDHDGDYKDHDIDYKDDDDKGAAHHHHHH

SEQ ID NO: 343 - protein, 304 aa, synthetic construct
  REGION 1..304: note = Nanobody sequence
EVQLVESGGGLVQPGGSLRLSCVASGDVHKINFLGWYRQAPGKEREKVAHISIGDQTDYADSAKGRFTISRDESKNMVYLQMNSLKPEDTAVYFCRAFSRIYPYDYWGQGTLVTVSSGGGGSGGGGSGGGGSGGGGSGGGGSGGGGSGGGGSEVQLVESGGGLVQAGGSLRLSCAASGITFSINTMGWYRQAPGKQRELVALISSIGDTYYADSVKGRFTISRDNAKNTVYLQMNSLKPEDTAVYYCKRFRTAAQGTDYWGQGTLVTVSSGAADYKDHDGDYKDHDIDYKDDDDKGAAHHHHHH

SEQ ID NO: 344 - protein, 171 aa, Homo sapiens
MEHSTFLSGLVLATLLSQVSPFKIPIEELEDRVFVNCNTSITWVEGTVGTLLSDITRLDLGKRILDPRGIYRCNGTDIYKDKESTVQVHYRMCQSCVELDPATVAGIIVTDVIATLLLALGVFCFAGHETGRLSGAADTQALLRNDQVYQPLRDRDDAQYSHLGGNWARNK

SEQ ID NO: 345 - protein, 182 aa, Homo sapiens
MEQGKGLAVLILAIILLQGTLAQSIKGNHLVKVYDYQEDGSVLLTCDAEAKNITWFKDGKMIGFLTEDKKKWNLGSNAKDPRGMYQCKGSQNKSKPLQVYYRMCQNCIELNAATISGFLFAEIVSIFVLAVGVYFIAGQDGVRQSRASDKQTLLPNDQLYQPLKDREDDQYSHLQGNQLRRN

SEQ ID NO: 346 - protein, 207 aa, Homo sapiens
MQSGTHWRVLGLCLLSVGVWGQDGNEEMGGITQTPYKVSISGTTVILTCPQYPGSEILWQHNDKNIGGDEDDKNIGSDEDHLSLKEFSELEQSGYYVCYPRGSKPEDANFYLYLRARVCENCMEMDVMSVATIVIVDICITGGLLLLVYYWSKNRKAKAKPVTRGAGAGGRQRGQNKERPPPVPNPDYEPIRKGQRDLYSGLNQRRI

SEQ ID NO: 347 - protein, 164 aa, Homo sapiens
MKWKALFTAAILQAQLPITEAQSFGLLDPKLCYLLDGILFIYGVILTALFLRVKFSRSADAPAYQQGQNQLYNELNLGRREEYDVLDKRRGRDPEMGGKPQRRKNPQEGLYNELQKDKMAEAYSEIGMKGERRRGKGHDGLYQGLSTATKDTYDALHMQALPPR

SEQ ID NO: 348 - protein, 142 aa, Homo sapiens
PNIQNPDPAVYQLRDSKSSDKSVCLFTDFDSQTNVSQSKDSDVYITDKTVLDMRSMDFKSNSAVAWSNKSDFACANAFNNSIIPEDTFFPSPESSCDVKLVEKSFETDTNFRILLLKVAGFNLLMTLRLWSSLNFQNLSVIG

SEQ ID NO: 349 - protein, 177 aa, Homo sapiens
EDLNKVFPPEVAVFEPSEAEISHTQKATLVCLATGFFPDHVELSWWVNGKEVHSGVSTDPQPLKEQPALNDSRYCLSSRLRVSATFWQNPRNHFRCQVQFYGLSENDEWTVSAEAWGRADCGFTSVSYQQGVLSATILYEILLGKATLYAVLVSALVLMAMVKRKDFQDRAKPVTQI

SEQ ID NO: 350 - protein, 118 aa, synthetic construct
  REGION 1..118: note = Nanobody sequence
EVQLVESGGGLVQAGGSLRLSCAASGITFSINTMGWYRQAPGKQRELVALISSIGDTYYADSVKGRFTISRDNAKNTVYLQMNSLKPEDTAVYYCKRFRTAAQGTDYWGQGTLVTVSS

SEQ ID NO: 351 - protein, 119 aa, synthetic construct
  REGION 1..119: note = Nanobody sequence
EVQLVESGGGLVQPGGSLRLSCAASGSIFGFNDMAWYRQAPGKQRELVALISRVGVTSSADSVKGRFTISRVNAKDTVYLQMNSLKPEDTAVYYCYMDQRLDGSTLAYWGQGTQVTVSS

SEQ ID NO: 352 - protein, 127 aa, synthetic construct
  REGION 1..127: note = Nanobody sequence
EVQLVESGGGLVQAGGSLRLSCAASGRTFSSYAMGWFRQAPGKEREFVVAINWSSGSTYYADSVKGRFTISRDNAKNTMYLQMNSLKPEDTAVYYCAAGYQINSGNYNFKDYEYDYWGQGTQVTVSS

SEQ ID NO: 353 - protein, 123 aa, synthetic construct
  REGION 1..123: note = Nanobody sequence
EVQLVESGGGSVQAGGSLRLSCAASGDTYGSYWMGWFRQAPGKEREGVAAINRGGGYTVYADSVKGRFTISRDTAKNTVYLQMNSLRPDDTADYYCAASGVLGGLHEDWFNYWGQGTLVTVSS

SEQ ID NO: 354 - protein, 123 aa, synthetic construct
  REGION 1..123: note = Nanobody sequence
EVQLVESGGGSVQAGGSLRLSCAASGDTYGSYWMGWFRQAPGQEREAVAAINRGGGYTVYADSVKGRFTISRDNAKNTLYLQMNSLRPDDTADYYCAASGVLGGLHEDWFNYWGQGTLVTVSS

SEQ ID NO: 355 - protein, 124 aa, synthetic construct
  REGION 1..124: note = Nanobody sequence
EVQLVESGGGSVQTGGSLRLTCAASGRTSRSYGMGWFRQAPGKEREFVSGISWRGDSTGYADSVKGRFTISRDNAKNTVDLQMNSLKPEDTAIYYCAAAAGSAWYGTLYEYDYWGQGTLVTVSS

SEQ ID NO: 356 - protein, 124 aa, synthetic construct
  REGION 1..124: note = Nanobody sequence
EVQLVESGGGSVQAGGSLRLTCAASGSTSRSYGMGWFRQAPGKEREFVSGISWRGDSTGYADSVKGRFTISRDNAKNTVDLQMNSLKPEDTAIYYCAAAAGSTWYGTLYEYDYWGQGTLVTVSS

SEQ ID NO: 357 - protein, 120 aa, synthetic construct
  REGION 1..120: note = Nanobody sequence
EVQLVESGGGLVQPGGSLRLSCTFSGGTFSSYTMGWFRQAPGKEREFVAEVRWGGVTTYSNSLKDRFSISEDSVKNAVYLQMNSLKPEDTAVYYCAAVRQMYMTVVPDYWGQGTLVTVSS

SEQ ID NO: 358 - protein, 129 aa, synthetic construct
  REGION 1..129: note = Nanobody sequence
EVQLVESGGGLVQAGGSLRLSCAASGRTFSSYVMGWFRQATGKEREFVATIAWDSGSTYYADSVKGRFTISRDNAKNTVHLQMNSLKPEDTAVYYCAASYNVYYNNYYYPISRDEYDYWGQGTLVTVSS

SEQ ID NO: 359 - protein, 133 aa, synthetic construct
  REGION 1..133: note = Nanobody sequence
DVQLQASGGGSVQAGGSLRLSCAASGYTIGPYCMGWFRQAPGKEREGVAAINMGGGITYYADSVKGRFTISQDNAKNTVYLLMNSLEPEDTAIYYCAADSTIYASYYECGHGLSTGGYGYDSWGQGTQVTVSS

SEQ ID NO: 360 - protein, 127 aa, synthetic construct
  REGION 1..127: note = Nanobody sequence
EVQLVESGGGLVQAGDSLRLSCAASGRTFSSYAMGWFRQAPGKEREFVAAISWSDGSTYYADSVKGRFTISRDNAKNTVYLQMNSLKPEDTAVYYCAADLTSTNPGSYIYIWAYDYWGQGTQVTVSS

SEQ ID NO: 361 - protein, 10 aa, synthetic construct
  REGION 1..10: note = CDR1
GDTYGSYWMG

SEQ ID NO: 362 - protein, 10 aa, synthetic construct
  REGION 1..10: note = CDR1
GGTFSSYTMG

SEQ ID NO: 363 - protein, 10 aa, synthetic construct
  REGION 1..10: note = CDR2
AINRGGGYTV

SEQ ID NO: 364 - protein, 9 aa, synthetic construct
  REGION 1..9: note = CDR2
EVRWGGVTT

SEQ ID NO: 365 - protein, 14 aa, synthetic construct
  REGION 1..14: note = CDR3
SGVLGGLHEDWFNY

SEQ ID NO: 366 - protein, 12 aa, synthetic construct
  REGION 1..12: note = CDR3
VRQMYMTVVPDY

SEQ ID NO: 367 - protein, 25 aa, synthetic construct
  REGION 1..25: note = FR1
EVQLVESGGGSVQAGGSLRLSCAAS

SEQ ID NO: 368 - protein, 25 aa, synthetic construct
  REGION 1..25: note = FR1
EVQLVESGGGLVQPGGSLRLSCTFS

SEQ ID NO: 369 - protein, 14 aa, synthetic construct
  REGION 1..14: note = FR2
WFRQAPGKEREGVA

SEQ ID NO: 370 - protein, 14 aa, synthetic construct
  REGION 1..14: note = FR2
WFRQAPGQEREAVA

SEQ ID NO: 371 - protein, 14 aa, synthetic construct
  REGION 1..14: note = FR2
WFRQAPGKEREFVA

SEQ ID NO: 372 - protein, 39 aa, synthetic construct
  REGION 1..39: note = FR3
YADSVKGRFTISRDTAKNTVYLQMNSLRPDDTADYYCAA

SEQ ID NO: 373 - protein, 39 aa, synthetic construct
  REGION 1..39: note = FR3
YADSVKGRFTISRDNAKNTLYLQMNSLRPDDTADYYCAA

SEQ ID NO: 374 - protein, 39 aa, synthetic construct
  REGION 1..39: note = FR3
YSNSLKDRFSISEDSVKNAVYLQMNSLKPEDTAVYYCAA

SEQ ID NO: 375 - protein, 11 aa, synthetic construct
  REGION 1..11: note = FR4
WGQGTLVTVSS

SEQ ID NO: 376 - protein, 5 aa, synthetic construct
  REGION 1..5: note = Linker
GGGGS

SEQ ID NO: 377 - protein, 7 aa, synthetic construct
  REGION 1..7: note = Linker
SGGSGGS

SEQ ID NO: 378 - protein, 9 aa, synthetic construct
  REGION 1..9: note = Linker
GGGGSGGGS

SEQ ID NO: 379 - protein, 10 aa, synthetic construct
  REGION 1..10: note = Linker
GGGGSGGGGS

SEQ ID NO: 380 - protein, 15 aa, synthetic construct
  REGION 1..15: note = Linker
GGGGSGGGGSGGGGS

SEQ ID NO: 381 - protein, 18 aa, synthetic construct
  REGION 1..18: note = Linker
GGGGSGGGGSGGGGGGGS

SEQ ID NO: 382 - protein, 20 aa, synthetic construct
  REGION 1..20: note = Linker
GGGGSGGGGSGGGGSGGGGS

SEQ ID NO: 383 - protein, 25 aa, synthetic construct
  REGION 1..25: note = Linker
GGGGSGGGGSGGGGSGGGGSGGGGS

SEQ ID NO: 384 - protein, 30 aa, synthetic construct
  REGION 1..30: note = Linker
GGGGSGGGGSGGGGSGGGGSGGGGSGGGGS

SEQ ID NO: 385 - protein, 35 aa, synthetic construct
  REGION 1..35: note = Linker
GGGGSGGGGSGGGGSGGGGSGGGGSGGGGSGGGGS

SEQ ID NO: 386 - skipped

SEQ ID NO: 387 - protein, 423 aa, synthetic construct
  REGION 1..423: note = Nanobody sequence
DVQLVESGGGLVQPGGSLRLSCTFSGGTFSSYTMGWFRQAPGKEREFVAEVRWGGVTTYSNSLKDRFSISEDSVKNAVYLQMNSLKPEDTAVYYCAAVRQMYMTVVPDYWGQGTLVTVSSGGGGSGGGGSGGGGSGGGGSGGGGSGGGGSGGGGSEVQLVESGGGLVQPGGSLRLSCAASGDVHKINILGWYRQAPAKEREMVAHITIGDATDYADSAKGRFTISRDEAKNMVYLQMNSLKPEDTAVYFCRAYSRIYPYNYWGQGTLVTVSSGGGGSGGGGSGGGGSGGGGSGGGGSGGGGSGGGGSEVQLVESGGGLVQPGNSLRLSCAASGFTFSSFGMSWVRQAPGKGLEWVSSISGSGSDTLYADSVKGRFTISRDNAKTTLYLQMNSLRPEDTAVYYCTIGGSLSRSSQGTLVTVSSA

SEQ ID NO: 388 - protein, 273 aa, synthetic construct
  REGION 1..273: note = Nanobody sequence
DVQLVESGGGLVQPGGSLRLSCTFSGGTFSSYTMGWFRQAPGKEREFVAEVRWGGVTTYSNSLKDRFSISEDSVKNAVYLQMNSLKPEDTAVYYCAAVRQMYMTVVPDYWGQGTLVTVSSGGGGSGGGGSGGGGSGGGGSGGGGSGGGGSGGGGSEVQLVESGGGLVQPGGSLRLSCVASGDVHKINFLGWYRQAPGKEREKVAHISIGDQTDYADSAKGRFTISRDESKNMVYLQMNSLKPEDTAVYFCRAFSRIYPYDYWGQGTLVTVSSA

SEQ ID NO: 389 - protein, 430 aa, synthetic construct
  REGION 1..430: note = Nanobody sequence
DVQLVESGGGLVQAGDSLRLSCAASGRTFSSYAMGWFRQAPGKEREFVAAISWSDGSTYYADSVKGRFTISRDNAKNTVYLQMNSLKPEDTAVYYCAADLTSTNPGSYIYIWAYDYWGQGTQVTVSSGGGGSGGGGSGGGGSGGGGSGGGGSGGGGSGGGGSEVQLVESGGGLVQPGGSLRLSCAASGDVHKINILGWYRQAPAKEREMVAHITIGDATDYADSAKGRFTISRDEAKNMVYLQMNSLKPEDTAVYFCRAYSRIYPYNYWGQGTLVTVSSGGGGSGGGGSGGGGSGGGGSGGGGSGGGGSGGGGSEVQLVESGGGLVQPGNSLRLSCAASGFTFSSFGMSWVRQAPGKGLEWVSSISGSGSDTLYADSVKGRFTISRDNAKTTLYLQMNSLRPEDTAVYYCTIGGSLSRSSQGTLVTVSSA

SEQ ID NO: 390 - protein, 473 aa, synthetic construct
  REGION 1..473: note = Nanobody sequence
EVQLVESGGGLVQAGGSLRLSCAASGRTFSSYVMGWFRQATGKEREFVATIAWDSGSTYYADSVKGRFTISRDNAKNTVHLQMNSLKPEDTAVYYCAASYNVYYNNYYYPISRDEYDYWGQGTLVTVSSGGGGSGGGGSGGGGSGGGGSGGGGSGGGGSGGGGSEVQLVESGGGSVQAGGSLRLSCAASGDTYGSYWMGWFRQAPGKEREGVAAINRGGGYTVYADSVKGRFTISRDTAKNTVYLQMNSLRPDDTADYYCAASGVLGGLHEDWFNYWGQGTLVTVSSGGGGSGGGGSGGGGSGGGGSGGGGSGGGGSGGGGSEVQLVESGGGLVQPGGSLRLSCVASGDVHKINFLGWYRQAPGKEREKVAHISIGDQTDYADSAKGRFTISRDESKNMVYLQMNSLKPEDTAVYFCRAFSRIYPYDYWGQGTLVTVSSGAADYKDHDGDYKDHDIDYKDDDDKGAAHHHHHH

SEQ ID NO: 391 - protein, 477 aa, synthetic construct
  REGION 1..477: note = Nanobody sequence
EVQLVESGGGSVQAGGSLRLSCAASGYTIGPYCMGWFRQAPGKEREGVAAINMGGGITYYADSVKGRFTISQDNAKNTVYLLMNSLEPEDTAIYYCAADSTIYASYYECGHGLSTGGYGYDSWGQGTLVTVSSGGGGSGGGGSGGGGSGGGGSGGGGSGGGGSGGGGSEVQLVESGGGSVQAGGSLRLSCAASGDTYGSYWMGWFRQAPGKEREGVAAINRGGGYTVYADSVKGRFTISRDTAKNTVYLQMNSLRPDDTADYYCAASGVLGGLHEDWFNYWGQGTLVTVSSGGGGSGGGGSGGGGSGGGGSGGGGSGGGGSGGGGSEVQLVESGGGLVQPGGSLRLSCVASGDVHKINFLGWYRQAPGKEREKVAHISIGDQTDYADSAKGRFTISRDESKNMVYLQMNSLKPEDTAVYFCRAFSRIYPYDYWGQGTLVTVSSGAADYKDHDGDYKDHDIDYKDDDDKGAAHHHHHH

SEQ ID NO: 392 - protein, 483 aa, synthetic construct
  REGION 1..483: note = Nanobody sequence
EVQLVESGGGLVQAGGSLRLSCAASGRTFSSYVMGWFRQATGKEREFVATIAWDSGSTYYADSVKGRFTISRDNAKNTVHLQMNSLKPEDTAVYYCAASYNVYYNNYYYPISRDEYDYWGQGTLVTVSSGGGGSGGGGSGGGGSGGGGSGGGGSGGGGSGGGGSEVQLVESGGGSVQAGGSLRLSCAASGYTIGPYCMGWFRQAPGKEREGVAAINMGGGITYYADSVKGRFTISQDNAKNTVYLLMNSLEPEDTAIYYCAADSTIYASYYECGHGLSTGGYGYDSWGQGTLVTVSSGGGGSGGGGSGGGGSGGGGSGGGGSGGGGSGGGGSEVQLVESGGGLVQPGGSLRLSCVASGDVHKINFLGWYRQAPGKEREKVAHISIGDQTDYADSAKGRFTISRDESKNMVYLQMNSLKPEDTAVYFCRAFSRIYPYDYWGQGTLVTVSSGAADYKDHDGDYKDHDIDYKDDDDKGAAHHHHHH

SEQ ID NO: 393 - protein, 107 aa, Homo sapiens
IQVEQSPPDLILQEGANSTLRCNFSDSVNNLQWFHQNPWGQLINLFYIPSGTKQNGRLSATTVATERYSLLYISSSQTTDSGVYFCAALIQGAQKLVFGQGTRLTIN

SEQ ID NO: 394 - protein, 108 aa, Homo sapiens
QLLEQSPQFLSIQEGENLTVYCNSSSVFSSLQWYRQEPGEGPVLLVTVVTGGEVKKLKRLTFQFGDARKDSSLHITAAQPGDTGLYLCAGAGSQGNLIFGKGTKLSVK

SEQ ID NO: 395 - protein, 110 aa, Homo sapiens
GDAKTTQPNSMESNEEEPVHLPCNHSTISGTDYIHWYRQLPSQGPEYVIHGLTSNVNNRMASLAIAEDRKSSTLILHRATLRDAAVYYCTVYGGATNKLIFGTGTLLAVQ

SEQ ID NO: 396 - protein, 96 aa, Macaca fascicularis
PYIQNPDPAVYQLRGSKSNDTSVCLFTDFDSVMNVSQSKDSDVHITDKTVLDMRSMDFKSNGAVAWSNKSDFACTSAFKDSVIPADTFFPSPESSC

SEQ ID NO: 397 - protein, 131 aa, Macaca mulatta
EDLKKVFPPKVAVFEPSEAEISHTQKATLVCLATGFYPDHVELSWWVNGKEVHSGVSTDPQPLKEQPALEDSRYSLSSRLRVSATFWHNPRNHFRCQVQFYGLSEDDEWTEDRDKPITQKISAEAWGRADC

SEQ ID NO: 398 - protein, 107 aa, Macaca mulatta
QQIMQIPQYQHVQEGEDFTTYCNSSTTLSNIQWYKQRPGGHPVFLIMLVKSGEVKKQKRLIFQFGEAKKNSSLHITATQTTDVGTYFCATTGVNNLFFGTGTRLTVL

SEQ ID NO: 399 - protein, 118 aa, Macaca mulatta
AGPVNAGVTQTPKFQVLKTGQSMTLQCAQDMNHDYMYWYRQDPGMGLRLIHYSVGEGSTEKGEVPDGYNVTRSNTEDFPLRLESAAPSQTSVYFCASSYWTGRSYEQYFGPGTRLTVI

SEQ ID NO: 400 - protein, 115 aa, synthetic construct [sequence omitted]

SEQ ID NO: 401 - protein, 115 aa, synthetic construct [sequence omitted]

SEQ ID NO: 402 - protein, 116 aa, synthetic construct
  REGION 1..116: note = Nanobody sequence
EVQLVESGGGVVQPGNSLRLSCAASGFTFSSFGMSWVRQAPGKGLEWVSSISGSGSDTLYADSVKGRFTISRDNAKTTLYLQMNSLRPEDTATYYCTIGGSLSRSSQGTLVTVSSA

SEQ ID NO: 403 - protein, 116 aa, synthetic construct
  REGION 1..116: note = Nanobody sequence
EVQLVESGGGVVQPGGSLRLSCAASGFTFRSFGMSWVRQAPGKGPEWVSSISGSGSDTLYADSVKGRFTISRDNSKNTLYLQMNSLRPEDTATYYCTIGGSLSRSSQGTLVTVSSA

SEQ ID NO: 404 - protein, 115 aa, synthetic construct [sequence omitted]

SEQ ID NO: 405 - protein, 116 aa, synthetic construct
  REGION 1..116: note = Nanobody sequence
EVQLVESGGGLVQPGNSLRLSCAASGFTFSSFGMSWVRQAPGKGLEWVSSISGSGSDTLYADSVKGRFTISRDNAKTTLYLQMNSLRPEDTAVYYCTIGGSLSRSSQGTLVKVSSA

SEQ ID NO: 406 - protein, 115 aa, synthetic construct
  REGION 1..115: note = Nanobody sequence
EVQLVESGGGVVQPGNSLRLSCAASGFTFSSFGMSWVRQAPGKGLEWVSSISGSGSDTLYADSVKGRFTISRDNAKTTLYLQMNSLRPEDTALYYCTIGGSLSRSSQGTLVTVSS

SEQ ID NO: 407 - protein, 116 aa, synthetic construct
  REGION 1..116: note = Nanobody sequence
EVQLVESGGGVVQPGNSLRLSCAASGFTFSSFGMSWVRQAPGKGLEWVSSISGSGSDTLYADSVKGRFTISRDNAKTTLYLQMNSLRPEDTALYYCTIGGSLSRSSQGTLVTVSSA

SEQ ID NO: 408 - protein, 117 aa, synthetic construct
  REGION 1..117: note = Nanobody sequence
EVQLVESGGGVVQPGNSLRLSCAASGFTFSSFGMSWVRQAPGKGLEWVSSISGSGSDTLYADSVKGRFTISRDNAKTTLYLQMNSLRPEDTALYYCTIGGSLSRSSQGTLVTVSSAA

SEQ ID NO: 409 - protein, 118 aa, synthetic construct
  REGION 1..118: note = Nanobody sequence
EVQLVESGGGVVQPGNSLRLSCAASGFTFSSFGMSWVRQAPGKGLEWVSSISGSGSDTLYADSVKGRFTISRDNAKTTLYLQMNSLRPEDTALYYCTIGGSLSRSSQGTLVTVSSAAA

SEQ ID NO: 410 - protein, 116 aa, synthetic construct
  REGION 1..116: note = Nanobody sequence
EVQLVESGGGVVQPGNSLRLSCAASGFTFSSFGMSWVRQAPGKGLEWVSSISGSGSDTLYADSVKGRFTISRDNAKTTLYLQMNSLRPEDTALYYCTIGGSLSRSSQGTLVTVSSG

SEQ ID NO: 411 - protein, 117 aa, synthetic construct
  REGION 1..117: note = Nanobody sequence
EVQLVESGGGVVQPGNSLRLSCAASGFTFSSFGMSWVRQAPGKGLEWVSSISGSGSDTLYADSVKGRFTISRDNAKTTLYLQMNSLRPEDTALYYCTIGGSLSRSSQGTLVTVSSGG

SEQ ID NO: 412 - protein, 118 aa, synthetic construct
  REGION 1..118: note = Nanobody sequence
EVQLVESGGGVVQPGNSLRLSCAASGFTFSSFGMSWVRQAPGKGLEWVSSISGSGSDTLYADSVKGRFTISRDNAKTTLYLQMNSLRPEDTALYYCTIGGSLSRSSQGTLVTVSSGGG

SEQ ID NO: 413 - protein, 293 aa, synthetic construct
  REGION 1..293: note = Nanobody sequence
EVQLVESGGGLVQGGGSLSLSCAASGRTFSSYAMAWFRQPPGKEREFVASISWSGENTNYRNSVKGRFTISRDNAKNTVYLQMNSLKPEDTAVYYCAAKIAKTYPDNWYWTKSNNYNYWGQGTLVTVSSGGGGSGGGGSGGGGSGGGGSGGGGSGGGGSGGGGSEVQLVESGGGLVQGGGSLSLSCAASGRTFSSYAMAWFRQPPGKEREFVASISWSGENTNYRNSVKGRFTISRDNAKNTVYLQMNSLKPEDTAVYYCAAKIAKTYPDNWYWTKSNNYNYWGQGTLVTVSS

SEQ ID NO: 414 - protein, 242 aa, synthetic construct
  REGION 1..242: note = Nanobody sequence
EVQLVESGGGLVQPGGSLRLSCTFSGGTFSSYTMGWFRQAPGKEREFVAEVRWGGVTTYSNSLKDRFSISEDSVKNAVYLQMNSLKPEDTAVYYCAAVRQMYMTVVPDYWGQGTLVTVSSGGGGSEVQLVESGGGLVQPGGSLRLSCAASGSVHKINFLGWYRQAPGKERGLVATITIGDTTDYADYAKGRFTISRDEARNMVYLQMNSLKPEDTAVYFCRAGSRLYPYNYWGQGTLVTVSS

SEQ ID NO: 415 - protein, 255 aa, synthetic construct
  REGION 1..255: note = Nanobody sequence
EVQLQASGGGSVQAGGSLRLSCAASGYTIGPYCMGWFRQAPGKEREGVAAINMGGGITYYADSVKGRFTISQDNAKNTVYLLMNSLEPEDTAIYYCAADSTIYASYYECGHGLSTGGYGYDSWGQGTQVTVSSGGGGSEVQLVESGGGLVQPGGSLRLSCAASGSVHKINFLGWYRQAPGKERGLVATITIGDTTDYADYAKGRFTISRDEARNMVYLQMNSLKPEDTAVYFCRAGSRLYPYNYWGQGTLVTVSS

SEQ ID NO: 416 - protein, 258 aa, synthetic construct
  REGION 1..258: note = Nanobody sequence
EVQLVESGGGLVQPGGSLRLSCTFSGGTFSSYTMGWFRQAPGKEREFVAEVRWGGVTTYSNSLKDRFSISEDSVKNAVYLQMNSLKPEDTAVYYCAAVRQMYMTVVPDYWGQGTLVTVSSGGGGSDVQLQASGGGSVQAGGSLRLSCAASGYTIGPYCMGWFRQAPGKEREGVAAINMGGGITYYADSVKGRFTISQDNAKNTVYLLMNSLEPEDTAIYYCAADSTIYASYYECGHGLSTGGYGYDSWGQGTQVTVSS

SEQ ID NO: 417 - protein, 242 aa, synthetic construct
  REGION 1..242: note = Nanobody sequence
EVQLVESGGGLVQPGGSLRLSCAASGSVHKINFLGWYRQAPGKERGLVATITIGDTTDYADYAKGRFTISRDEARNMVYLQMNSLKPEDTAVYFCRAGSRLYPYNYWGQGTLVTVSSGGGGSEVQLVESGGGLVQPGGSLRLSCTFSGGTFSSYTMGWFRQAPGKEREFVAEVRWGGVTTYSNSLKDRFSISEDSVKNAVYLQMNSLKPEDTAVYYCAAVRQMYMTVVPDYWGQGTLVTVSS

SEQ ID NO: 418 - protein, 246 aa, synthetic construct
  REGION 1..246: note = Nanobody sequence
EVQLVESGGGLVQPGGSLRLSCTFSGGTFSSYTMGWFRQAPGKEREFVAEVRWGGVTTYSNSLKDRFSISEDSVKNAVYLQMNSLKPEDTAVYYCAAVRQMYMTVVPDYWGQGTLVTVSSGGGGSGGGSEVQLVESGGGLVQPGGSLRLSCAASGSVHKINFLGWYRQAPGKERGLVATITIGDTTDYADYAKGRFTISRDEARNMVYLQMNSLKPEDTAVYFCRAGSRLYPYNYWGQGTLVTVSS

SEQ ID NO: 419 - protein, 259 aa, synthetic construct
  REGION 1..259: note = Nanobody sequence
EVQLQASGGGSVQAGGSLRLSCAASGYTIGPYCMGWFRQAPGKEREGVAAINMGGGITYYADSVKGRFTISQDNAKNTVYLLMNSLEPEDTAIYYCAADSTIYASYYECGHGLSTGGYGYDSWGQGTQVTVSSGGGGSGGGSEVQLVESGGGLVQPGGSLRLSCAASGSVHKINFLGWYRQAPGKERGLVATITIGDTTDYADYAKGRFTISRDEARNMVYLQMNSLKPEDTAVYFCRAGSRLYPYNYWGQGTLVTVSS

SEQ ID NO: 420 - protein, 262 aa, synthetic construct
  REGION 1..262: note = Nanobody sequence
EVQLVESGGGLVQPGGSLRLSCTFSGGTFSSYTMGWFRQAPGKEREFVAEVRWGGVTTYSNSLKDRFSISEDSVKNAVYLQMNSLKPEDTAVYYCAAVRQMYMTVVPDYWGQGTLVTVSSGGGGSGGGSDVQLQASGGGSVQAGGSLRLSCAASGYTIGPYCMGWFRQAPGKEREGVAAINMGGGITYYADSVKGRFTISQDNAKNTVYLLMNSLEPEDTAIYYCAADSTIYASYYECGHGLSTGGYGYDSWGQGTQVTVSS

SEQ ID NO: 421 - protein, 246 aa, synthetic construct
  REGION 1..246: note = Nanobody sequence
EVQLVESGGGLVQPGGSLRLSCAASGSVHKINFLGWYRQAPGKERGLVATITIGDTTDYADYAKGRFTISRDEARNMVYLQMNSLKPEDTAVYFCRAGSRLYPYNYWGQGTLVTVSSGGGGSGGGSEVQLVESGGGLVQPGGSLRLSCTFSGGTFSSYTMGWFRQAPGKEREFVAEVRWGGVTTYSNSLKDRFSISEDSVKNAVYLQMNSLKPEDTAVYYCAAVRQMYMTVVPDYWGQGTLVTVSS

SEQ ID NO: 422 - protein, 272 aa, synthetic construct
  REGION 1..272: note = Nanobody sequence
EVQLVESGGGLVQPGGSLRLSCTFSGGTFSSYTMGWFRQAPGKEREFVAEVRWGGVTTYSNSLKDRFSISEDSVKNAVYLQMNSLKPEDTAVYYCAAVRQMYMTVVPDYWGQGTLVTVSSGGGGSGGGGSGGGGSGGGGSGGGGSGGGGSGGGGSEVQLVESGGGLVQPGGSLRLSCAASGSVHKINFLGWYRQAPGKERGLVATITIGDTTDYADYAKGRFTISRDEARNMVYLQMNSLKPEDTAVYFCRAGSRLYPYNYWGQGTLVTVSS

SEQ ID NO: 423 - protein, 285 aa, synthetic construct
  REGION 1..285: note = Nanobody sequence
EVQLQASGGGSVQAGGSLRLSCAASGYTIGPYCMGWFRQAPGKEREGVAAINMGGGITYYADSVKGRFTISQDNAKNTVYLLMNSLEPEDTAIYYCAADSTIYASYYECGHGLSTGGYGYDSWGQGTQVTVSSGGGGSGGGGSGGGGSGGGGSGGGGSGGGGSGGGGSEVQLVESGGGLVQPGGSLRLSCAASGSVHKINFLGWYRQAPGKERGLVATITIGDTTDYADYAKGRFTISRDEARNMVYLQMNSLKPEDTAVYFCRAGSRLYPYNYWGQGTLVTVSS

SEQ ID NO: 424 - protein, 288 aa, synthetic construct
  REGION 1..288: note = Nanobody sequence
EVQLVESGGGLVQPGGSLRLSCTFSGGTFSSYTMGWFRQAPGKEREFVAEVRWGGVTTYSNSLKDRFSISEDSVKNAVYLQMNSLKPEDTAVYYCAAVRQMYMTVVPDYWGQGTLVTVSSGGGGSGGGGSGGGGSGGGGSGGGGSGGGGSGGGGSDVQLQASGGGSVQAGGSLRLSCAASGYTIGPYCMGWFRQAPGKEREGVAAINMGGGITYYADSVKGRFTISQDNAKNTVYLLMNSLEPEDTAIYYCAADSTIYASYYECGHGLSTGGYGYDSWGQGTQVTVSS

SEQ ID NO: 425 - protein, 272 aa, synthetic construct
  REGION 1..272: note = Nanobody sequence
EVQLVESGGGLVQPGGSLRLSCAASGSVHKINFLGWYRQAPGKERGLVATITIGDTTDYADYAKGRFTISRDEARNMVYLQMNSLKPEDTAVYFCRAGSRLYPYNYWGQGTLVTVSSGGGGSGGGGSGGGGSGGGGSGGGGSGGGGSGGGGSEVQLVESGGGLVQPGGSLRLSCTFSGGTFSSYTMGWFRQAPGKEREFVAEVRWGGVTTYSNSLKDRFSISEDSVKNAVYLQMNSLKPEDTAVYYCAAVRQMYMTVVPDYWGQGTLVTVSS

SEQ ID NO: 426 - protein, 288 aa, synthetic construct
  REGION 1..288: note = Nanobody sequence
EVQLQASGGGSVQAGGSLRLSCAASGYTIGPYCMGWFRQAPGKEREGVAAINMGGGITYYADSVKGRFTISQDNAKNTVYLLMNSLEPEDTAIYYCAADSTIYASYYECGHGLSTGGYGYDSWGQGTQVTVSSGGGGSGGGGSGGGGSGGGGSGGGGSGGGGSGGGGSEVQLVESGGGLVQPGGSLRLSCTFSGGTFSSYTMGWFRQAPGKEREFVAEVRWGGVTTYSNSLKDRFSISEDSVKNAVYLQMNSLKPEDTAVYYCAAVRQMYMTVVPDYWGQGTLVTVSS

SEQ ID NO: 427 - protein, 285 aa, synthetic construct
  REGION 1..285: note = Nanobody sequence
EVQLVESGGGLVQPGGSLRLSCAASGSVHKINFLGWYRQAPGKERGLVATITIGDTTDYADYAKGRFTISRDEARNMVYLQMNSLKPEDTAVYFCRAGSRLYPYNYWGQGTLVTVSSGGGGSGGGGSGGGGSGGGGSGGGGSGGGGSGGGGSDVQLQASGGGSVQAGGSLRLSCAASGYTIGPYCMGWFRQAPGKEREGVAAINMGGGITYYADSVKGRFTISQDNAKNTVYLLMNSLEPEDTAIYYCAADSTIYASYYECGHGLSTGGYGYDSWGQGTQVTVSS

SEQ ID NO: 428 - protein, 272 aa, synthetic construct
  REGION 1..272: note = Nanobody sequence
EVQLVESGGGLVQPGGSLRLSCAASGDVYKINFLGWHRQAPGKEREKVAHITIGDATDYADSAKGRFTISRDEAKNMVYLQMNSLKPEDTAVYFCRAGSRIYPYDYWGQGTLVTVSSGGGGSGGGGSGGGGSGGGGSGGGGSGGGGSGGGGSEVQLVESGGGLVQPGGSLRLSCTFSGGTFSSYTMGWFRQAPGKEREFVAEVRWGGVTTYSNSLKDRFSISEDSVKNAVYLQMNSLKPEDTAVYYCAAVRQMYMTVVPDYWGQGTLVTVSS

SEQ ID NO: 429 - protein, 272 aa, synthetic construct
  REGION 1..272: note = Nanobody sequence
EVQLVESGGGLVQPGGSLKLSCAASGAVHKINFLGWYRQTPEKEREMVATITIGDEVDYADSAKGRFTISRDEAKNMVYLQMTSLKPEDTAVYVCRAGSRLYPYNYWGQGTLVTVSSGGGGSGGGGSGGGGSGGGGSGGGGSGGGGSGGGGSEVQLVESGGGLVQPGGSLRLSCTFSGGTFSSYTMGWFRQAPGKEREFVAEVRWGGVTTYSNSLKDRFSISEDSVKNAVYLQMNSLKPEDTAVYYCAAVRQMYMTVVPDYWGQGTLVTVSS

SEQ ID NO: 430 - protein, 272 aa, synthetic construct
  REGION 1..272: note = Nanobody sequence
EVQLVESGGGLVQPGGSLRLSCITSGETFKINIWGWYRQAPGKQRELVASLTIGGATNYADSVKGRFTISEDSAKNTVYLQMNSLKPEDTAVYFCNAKSRLYPYDYWGQGTLVTVSSGGGGSGGGGSGGGGSGGGGSGGGGSGGGGSGGGGSEVQLVESGGGLVQPGGSLRLSCTFSGGTFSSYTMGWFRQAPGKEREFVAEVRWGGVTTYSNSLKDRFSISEDSVKNAVYLQMNSLKPEDTAVYYCAAVRQMYMTVVPDYWGQGTLVTVSS

SEQ ID NO: 431 - protein, 272 aa, synthetic construct
  REGION 1..272: note = Nanobody sequence
EVQLVESGGGLVQPGGSLRLSCAASGSVHLLNFLGWYRQAPGKEREMVAHITIADATDYAHFAKGRFTISRDEAKNMVYLQMNSLRPEDTAVYFCRAGSRIYPYDYWGQGTLVTVSSGGGGSGGGGSGGGGSGGGGSGGGGSGGGGSGGGGSEVQLVESGGGLVQPGGSLRLSCTFSGGTFSSYTMGWFRQAPGKEREFVAEVRWGGVTTYSNSLKDRFSISEDSVKNAVYLQMNSLKPEDTAVYYCAAVRQMYMTVVPDYWGQGTLVTVSS

SEQ ID NO: 432 - protein, 272 aa, synthetic construct
  REGION 1..272: note = Nanobody sequence
EVQLVESGGGLVQPGGSLRLSCITSGETFKINIWGWYRQAPGKQRELVASLTIGGATDYADSVKGRFTISEDSAKNTVYLQMNSLKAEDTAVYFCNAKSRLYPYDYWGQGTLVTVSSGGGGSGGGGSGGGGSGGGGSGGGGSGGGGSGGGGSEVQLVESGGGLVQPGGSLRLSCTFSGGTFSSYTMGWFRQAPGKEREFVAEVRWGGVTTYSNSLKDRFSISEDSVKNAVYLQMNSLKPEDTAVYYCAAVRQMYMTVVPDYWGQGTLVTVSS

SEQ ID NO: 433 - protein, 272 aa, synthetic construct
  REGION 1..272: note = Nanobody sequence
EVQLVESGGGLVQPGGSLRLSCAASGEVYKINFLGWYRQAPGKEREKVAHITIADAADYADFAKGRFTISRDEAKNMVYLQMNSLRPEDTAVYFCRAGSRIWPYDYWGQGTLVTVSSGGGGSGGGGSGGGGSGGGGSGGGGSGGGGSGGGGSEVQLVESGGGLVQPGGSLRLSCTFSGGTFSSYTMGWFRQAPGKEREFVAEVRWGGVTTYSNSLKDRFSISEDSVKNAVYLQMNSLKPEDTAVYYCAAVRQMYMTVVPDYWGQGTLVTVSS

SEQ ID NO: 434 - protein, 272 aa, synthetic construct
  REGION 1..272: note = Nanobody sequence
EVQLVESGGGLVQPGGSLRLSCVASGDVHKINFLGWYRQAPGKEREKVAHISIGDQTDYADSAKGRFTISRDESKNMVYLQMNSLKPEDTAVYFCRAFSRIYPYDYWGQGTLVTVSSGGGGSGGGGSGGGGSGGGGSGGGGSGGGGSGGGGSEVQLVESGGGLVQPGGSLRLSCTFSGGTFSSYTMGWFRQAPGKEREFVAEVRWGGVTTYSNSLKDRFSISEDSVKNAVYLQMNSLKPEDTAVYYCAAVRQMYMTVVPDYWGQGTLVTVSS

SEQ ID NO: 435 - protein, 272 aa, synthetic construct
  REGION 1..272: note = Nanobody sequence
EVQLVESGGGLVQPGGSLRLSCAASGEIGRINFYRWYRQAPGNQREVVATITIADKTDYADSAKGRFTISRDESRNMVYLQMSSLKPEDTAVYFCHAGSRLYPYDYWGQGTLVTVSSGGGGSGGGGSGGGGSGGGGSGGGGSGGGGSGGGGSEVQLVESGGGLVQPGGSLRLSCTFSGGTFSSYTMGWFRQAPGKEREFVAEVRWGGVTTYSNSLKDRFSISEDSVKNAVYLQMNSLKPEDTAVYYCAAVRQMYMTVVPDYWGQGTLVTVSS

SEQ ID NO: 436 - protein, 272 aa, synthetic construct
  REGION 1..272: note = Nanobody sequence
EVQLVESGGGLVQPGGSLRLSCVASGDVHKINFLGWYRQAPGKEREKVAHITIGDQADYADSAKGRFTISRDEAKNMVYLQMNSLKPEDTAVYFCRAGSRIYPYDYWGQGTLVTVSSGGGGSGGGGSGGGGSGGGGSGGGGSGGGGSGGGGSEVQLVESGGGLVQPGGSLRLSCTFSGGTFSSYTMGWFRQAPGKEREFVAEVRWGGVTTYSNSLKDRFSISEDSVKNAVYLQMNSLKPEDTAVYYCAAVRQMYMTVVPDYWGQGTLVTVSS

SEQ ID NO: 437 - protein, 272 aa, synthetic construct
  REGION 1..272: note = Nanobody sequence
EVQLVESGGGLVQPGGSLRLSCAASGDVHKINILGWYRQAPAKEREMVAHITIGDATDYADSAKGRFTISRDEAKNMVYLQMNSLKPEDTAVYFCRAYSRIYPYNYWGQGTLVTVSSGGGGSGGGGSGGGGSGGGGSGGGGSGGGGSGGGGSEVQLVESGGGLVQPGGSLRLSCTFSGGTFSSYTMGWFRQAPGKEREFVAEVRWGGVTTYSNSLKDRFSISEDSVKNAVYLQMNSLKPEDTAVYYCAAVRQMYMTVVPDYWGQGTLVTVSS

SEQ ID NO: 438 - protein, 272 aa, synthetic construct
  REGION 1..272: note = Nanobody sequence
EVQLVESGGGLVQPGGSLRLSCAASGSVHKINFLGWYRQAPGKERELVATITIGDTTDYADSAKGRFTISRDEAKNMVYLQMNSLKPEDTAVYFCRAGSRLYPYNYWGQGTLVTVSSGGGGSGGGGSGGGGSGGGGSGGGGSGGGGSGGGGSEVQLVESGGGLVQPGGSLRLSCTFSGGTFSSYTMGWFRQAPGKEREFVAEVRWGGVTTYSNSLKDRFSISEDSVKNAVYLQMNSLKPEDTAVYYCAAVRQMYMTVVPDYWGQGTLVTVSS

SEQ ID NO: 439 - protein, 272 aa, synthetic construct; identical to SEQ ID NO: 425
  REGION 1..272: note = Nanobody sequence

SEQ ID NO: 440 - protein, 272 aa, synthetic construct
  REGION 1..272: note = Nanobody sequence
EVQLVESGGGLVQPGGSLRLSCAASGDVHKINILGWYRQAPAKEREMVAHITIGDATDYADSAKGRFTISRDEAKNMVYLQMNSLKPEDTAVYLCRAYSRIYPYNYWGQGTLVTVSSGGGGSGGGGSGGGGSGGGGSGGGGSGGGGSGGGGSEVQLVESGGGLVQPGGSLRLSCTFSGGTFSSYTMGWFRQAPGKEREFVAEVRWGGVTTYSNSLKDRFSISEDSVKNAVYLQMNSLKPEDTAVYYCAAVRQMYMTVVPDYWGQGTLVTVSS

SEQ ID NO: 441 - protein, 272 aa, synthetic construct
  REGION 1..272: note = Nanobody sequence
EVQLVESGGGLVQPGGSLRLSCTFSGGTFSSYTMGWFRQAPGKEREFVAEVRWGGVTTYSNSLKDRFSISEDSVKNAVYLQMNSLKPEDTAVYYCAAVRQMYMTVVPDYWGQGTLVTVSSGGGGSGGGGSGGGGSGGGGSGGGGSGGGGSGGGGSEVQLVESGGGLVQPGGSLRLSCVASGDVHKINFLGWYRQAPGKEREKVAHISIGDQTDYADSAKGRFTISRDESKNMVYLQMNSLKPEDTAVYFCRAFSRIYPYDYWGQGTLVTVSS

SEQ ID NO: 442 - protein, 272 aa, synthetic construct
  REGION 1..272: note = Nanobody sequence
EVQLVESGGGLVQPGGSLRLSCTFSGGTFSSYTMGWFRQAPGKEREFVAEVRWGGVTTYSNSLKDRFSISEDSVKNAVYLQMNSLKPEDTAVYYCAAVRQMYMTVVPDYWGQGTLVTVSSGGGGSGGGGSGGGGSGGGGSGGGGSGGGGSGGGGSEVQLVESGGGLVQPGGSLRLSCAASGEIGRINFYRWYRQAPGNQREVVATITIADKTDYADSAKGRFTISRDESRNMVYLQMSSLKPEDTAVYFCHAGSRLYPYDYWGQGTLVTVSS

SEQ ID NO: 443 - protein, 272 aa, synthetic construct
  REGION 1..272: note = Nanobody sequence
EVQLVESGGGLVQPGGSLRLSCTFSGGTFSSYTMGWFRQAPGKEREFVAEVRWGGVTTYSNSLKDRFSISEDSVKNAVYLQMNSLKPEDTAVYYCAAVRQMYMTVVPDYWGQGTLVTVSSGGGGSGGGGSGGGGSGGGGSGGGGSGGGGSGGGGSEVQLVESGGGLVQPGGSLRLSCVASGDVHKINFLGWYRQAPGKEREKVAHITIGDQADYADSAKGRFTISRDEAKNMVYLQMNSLKPEDTAVYFCRAGSRIYPYDYWGQGTLVTVSS

SEQ ID NO: 444 - protein, 272 aa, synthetic construct
  REGION 1..272: note = Nanobody sequence
EVQLVESGGGLVQPGGSLRLSCTFSGGTFSSYTMGWFRQAPGKEREFVAEVRWGGVTTYSNSLKDRFSISEDSVKNAVYLQMNSLKPEDTAVYYCAAVRQMYMTVVPDYWGQGTLVTVSSGGGGSGGGGSGGGGSGGGGSGGGGSGGGGSGGGGSEVQLVESGGGLVQPGGSLRLSCAASGDVHKINILGWYRQAPAKEREMVAHITIGDATDYADSAKGRFTISRDEAKNMVYLQMNSLKPEDTAVYFCRAYSRIYPYNYWGQGTLVTVSS

SEQ ID NO: 445 - protein, 272 aa, synthetic construct
  REGION 1..272: note = Nanobody sequence
EVQLVESGGGLVQPGGSLRLSCTFSGGTFSSYTMGWFRQAPGKEREFVAEVRWGGVTTYSNSLKDRFSISEDSVKNAVYLQMNSLKPEDTAVYYCAAVRQMYMTVVPDYWGQGTLVTVSSGGGGSGGGGSGGGGSGGGGSGGGGSGGGGSGGGGSEVQLVESGGGLVQPGGSLRLSCAASGSVHKINFLGWYRQAPGKERELVATITIGDTTDYADSAKGRFTISRDEAKNMVYLQMNSLKPEDTAVYFCRAGSRLYPYNYWGQGTLVTVSS

SEQ ID NO: 446 - protein, 272 aa, synthetic construct; identical to SEQ ID NO: 422
  REGION 1..272: note = Nanobody sequence

SEQ ID NO: 447 - protein, 272 aa, synthetic construct
  REGION 1..272: note = Nanobody sequence
EVQLVESGGGLVQPGGSLRLSCTFSGGTFSSYTMGWFRQAPGKEREFVAEVRWGGVTTYSNSLKDRFSISEDSVKNAVYLQMNSLKPEDTAVYYCAAVRQMYMTVVPDYWGQGTLVTVSSGGGGSGGGGSGGGGSGGGGSGGGGSGGGGSGGGGSEVQLVESGGGLVQPGGSLRLSCAASGDVYKINFLGWHRQAPGKEREKVAHITIGDATDYADSAKGRFTISRDEAKNMVYLQMNSLKPEDTAVYFCRAGSRIYPYDYWGQGTLVTVSS

SEQ ID NO: 448 - protein, 272 aa, synthetic construct
  REGION 1..272: note = Nanobody sequence
EVQLVESGGGLVQPGGSLRLSCTFSGGTFSSYTMGWFRQAPGKEREFVAEVRWGGVTTYSNSLKDRFSISEDSVKNAVYLQMNSLKPEDTAVYYCAAVRQMYMTVVPDYWGQGTLVTVSSGGGGSGGGGSGGGGSGGGGSGGGGSGGGGSGGGGSEVQLVESGGGLVQPGGSLRLSCAASGEVYKINFLGWYRQAPGKEREKVAHITIADAADYADFAKGRFTISRDEAKNMVYLQMNSLRPEDTAVYFCRAGSRIWPYDYWGQGTLVTVSS

SEQ ID NO: 449 - protein, 272 aa, synthetic construct
  REGION 1..272: note = Nanobody sequence
EVQLVESGGGLVQPGGSLRLSCTFSGGTFSSYTMGWFRQAPGKEREFVAEVRWGGVTTYSNSLKDRFSISEDSVKNAVYLQMNSLKPEDTAVYYCAAVRQMYMTVVPDYWGQGTLVTVSSGGGGSGGGGSGGGGSGGGGSGGGGSGGGGSGGGGSEVQLVESGGDLVQPGGSLRLSCAASGDVHKINFLGWYRQAPGKEREMVAHITIADATDYAEFAKGRFTISRDEPKNMVYLQMNSLKPEDTAVYLCRAGSRIYPYNYWGQGTLVTVSS

SEQ ID NO: 450 - protein, 272 aa, synthetic construct
  REGION 1..272: note = Nanobody sequence
EVQLVESGGGLVQPGGSLRLSCTFSGGTFSSYTMGWFRQAPGKEREFVAEVRWGGVTTYSNSLKDRFSISEDSVKNAVYLQMNSLKPEDTAVYYCAAVRQMYMTVVPDYWGQGTLVTVSSGGGGSGGGGSGGGGSGGGGSGGGGSGGGGSGGGGSEVQLVESGGGLVQPGGSLRLSCITSGETFKINIWGWYRQAPGKQRELVASLTIGGATNYADSVKGRFTISEDSAKNTVYLQMNSLKPEDTAVYFCNAKSRLYPYDYWGQGTLVTVSS

SEQ ID NO: 451 - protein, 272 aa, synthetic construct
  REGION 1..272: note = Nanobody sequence
EVQLVESGGGLVQPGGSLRLSCTFSGGTFSSYTMGWFRQAPGKEREFVAEVRWGGVTTYSNSLKDRFSISEDSVKNAVYLQMNSLKPEDTAVYYCAAVRQMYMTVVPDYWGQGTLVTVSSGGGGSGGGGSGGGGSGGGGSGGGGSGGGGSGGGGSEVQLVESGGGLVQPGGSLRLSCAASGSVHLLNFLGWYRQAPGKEREMVAHITIADATDYAHFAKGRFTISRDEAKNMVYLQMNSLRPEDTAVYFCRAGSRIYPYDYWGQGTLVTVSS

SEQ ID NO: 452 - protein, 272 aa, synthetic construct
  REGION 1..272: note = Nanobody sequence
EVQLVESGGGLVQPGGSLRLSCTFSGGTFSSYTMGWFRQAPGKEREFVAEVRWGGVTTYSNSLKDRFSISEDSVKNAVYLQMNSLKPEDTAVYYCAAVRQMYMTVVPDYWGQGTLVTVSSGGGGSGGGGSGGGGSGGGGSGGGGSGGGGSGGGGSEVQLVESGGGLVQPGGSLRLSCITSGETFKINIWGWYRQAPGKQRELVASLTIGGATDYADSVKGRFTISEDSAKNTVYLQMNSLKAEDTAVYFCNAKSRLYPYDYWGQGTLVTVSS

SEQ ID NO: 453 - protein, 272 aa, synthetic construct
  REGION 1..272: note = Nanobody sequence
EVQLVESGGGLVQPGGSLRLSCAASGDVHKINILGWYRQAPAKEREMVAHITIGDATSYADSAKGRFTISRDEAKNMVYLQLNNLKPEDTAVYFCRAYSRIYPYNYWGQGTLVTVSSGGGGSGGGGSGGGGSGGGGSGGGGSGGGGSGGGGSEVQLVESGGGLVQPGGSLRLSCTFSGGTFSSYTMGWFRQAPGKEREFVAEVRWGGVTTYSNSLKDRFSISEDSVKNAVYLQMNSLKPEDTAVYYCAAVRQMYMTVVPDYWGQGTLVTVSS

SEQ ID NO: 454 - protein, 272 aa, synthetic construct; identical to SEQ ID NO: 434
  REGION 1..272: note = Nanobody sequence

SEQ ID NO: 455 - protein, 272 aa, synthetic construct
  REGION 1..272: note = Nanobody sequence
EVQLVESGGGLVQPGGSLRLSCTFSGGTFSSYTMGWFRQAPGKEREFVAEVRWGGVTTYSNSLKDRFSISEDSVKNAVYLQMNSLKPEDTAVYYCAAVRQMYMTVVPDYWGQGTLVTVSSGGGGSGGGGSGGGGSGGGGSGGGGSGGGGSGGGGSEVQLVESGGGLVQPGGSLRLSCAASGDVHKINILGWYRQAPAKEREMVAHITIGDATSYADSAKGRFTISRDEAKNMVYLQLNNLKPEDTAVYFCRAYSRIYPYNYWGQGTLVTVSS

SEQ ID NO: 456 - protein, 272 aa, synthetic construct; identical to SEQ ID NO: 441
  REGION 1..272: note = Nanobody sequence

SEQ ID NO: 457 - protein, 272 aa, synthetic construct
  REGION 1..272: note = Nanobody sequence
EVQLVESGGDLVQPGGSLRLSCAASGDVHKINFLGWYRQAPGKEREMVAHITIADATDYAEFAKGRFTISRDEPKNMVYLQMNSLKPEDTAVYLCRAGSRIYPYNYWGQGTLVTVSSGGGGSGGGGSGGGGSGGGGSGGGGSGGGGSGGGGSEVQLVESGGGLVQPGGSLRLSCTFSGGTFSSYTMGWFRQAPGKEREFVAEVRWGGVTTYSNSLKDRFSISEDSVKNAVYLQMNSLKPEDTAVYYCAAVRQMYMTVVPDYWGQGTLVTVSS

SEQ ID NO: 458 - protein, 272 aa, synthetic construct
  REGION 1..272: note = Nanobody sequence
EVQLVESGGGLVQPGGSLRLSCTFSGGTFSSYTMGWFRQAPGKEREFVAEVRWGGVTTYSNSLKDRFSISEDSVKNAVYLQMNSLKPEDTAVYYCAAVRQMYMTVVPDYWGQGTLVTVSSGGGGSGGGGSGGGGSGGGGSGGGGSGGGGSGGGGSEVQLVESGGGLVQPGGSLRLSCAASGDVHKINILGWYRQAPAKEREMVAHITIGDATDYADSAKGRFTISRDEAKNMVYLQMNSLKPEDTAVYLCRAYSRIYPYNYWGQGTLVTVSS

SEQ ID NO: 459 - protein, 272 aa, synthetic construct
  REGION 1..272: note = Nanobody sequence
EVQLVESGGGLVQPGGSLRLSCTFSGGTFSSYTMGWFRQAPGKEREFVAEVRWGGVTTYSNSLKDRFSISEDSVKNAVYLQMNSLKPEDTAVYYCAAVRQMYMTVVPDYWGQGTLVTVSSGGGGSGGGGSGGGGSGGGGSGGGGSGGGGSGGGGSEVQLVESGGGLVQPGGSLKLSCAASGAVHKINFLGWYRQTPEKEREMVATITIGDEVDYADSAKGRFTISRDEAKNMVYLQMTSLKPEDTAVYVCRAGSRLYPYNYWGQGTLVTVSS

SEQ ID NO: 460 - protein, 422 aa, synthetic construct
  REGION 1..422: note = Nanobody sequence
EVQLVESGGGLVQPGGSLRLSCTFSGGTFSSYTMGWFRQAPGKEREFVAEVRWGGVTTYSNSLKDRFSISEDSVKNAVYLQMNSLKPEDTAVYYCAAVRQMYMTVVPDYWGQGTLVTVSSGGGGSGGGGSGGGGSGGGGSGGGGSGGGGSGGGGSEVQLVESGGGLVQPGGSLRLSCVASGDVHKINFLGWYRQAPGKEREKVAHISIGDQTDYADSAKGRFTISRDESKNMVYLQMNSLKPEDTAVYFCRAFSRIYPYDYWGQGTLVTVSSGGGGSGGGGSGGGGSGGGGSGGGGSGGGGSGGGGSEVQLVESGGGLVQPGNSLRLSCAASGFTFSSFGMSWVRQAPGKGLEWVSSISGSGSDTLYADSVKGRFTISRDNAKTTLYLQMNSLRPEDTAVYYCTIGGSLSRSSQGTLVTVSS

SEQ ID NO: 461 - protein, 422 aa, synthetic construct
  REGION 1..422: note = Nanobody sequence
EVQLVESGGGLVQPGGSLRLSCTFSGGTFSSYTMGWFRQAPGKEREFVAEVRWGGVTTYSNSLKDRFSISEDSVKNAVYLQMNSLKPEDTAVYYCAAVRQMYMTVVPDYWGQGTLVTVSSGGGGSGGGGSGGGGSGGGGSGGGGSGGGGSGGGGSEVQLVESGGGLVQPGGSLRLSCITSGETFKINIWGWYRQAPGKQRELVASLTIGGATNYADSVKGRFTISEDSAKNTVYLQMNSLKPEDTAVYFCNAKSRLYPYDYWGQGTLVTVSSGGGGSGGGGSGGGGSGGGGSGGGGSGGGGSGGGGSEVQLVESGGGLVQPGNSLRLSCAASGFTFSSFGMSWVRQAPGKGLEWVSSISGSGSDTLYADSVKGRFTISRDNAKTTLYLQMNSLRPEDTAVYYCTIGGSLSRSSQGTLVTVSS

SEQ ID NO: 462 - protein, 270 aa, synthetic construct
  REGION 1..270: note = Nanobody sequence
EVQLVESGGGLVQAGGSLRLSCAASGITFSINTMGWYRQAPGKQRELVALISSIGDTYYADSVKGRFTISRDNAKNTVYLQMNSLKPEDTAVYYCKRFRTAAQGTDYWGQGTLVTVSSGGGGSGGGGSGGGGSGGGGSGGGGSGGGGSGGGGSEVQLVESGGGLVQPGGSLRLSCVASGDVHKINFLGWYRQAPGKEREKVAHISIGDQTDYADSAKGRFTISRDESKNMVYLQMNSLKPEDTAVYFCRAFSRIYPYDYWGQGTLVTVSS

SEQ ID NO: 463 - protein, 270 aa, synthetic construct
  REGION 1..270: note = Nanobody sequence
EVQLVESGGGLVQPGGSLRLSCVASGDVHKINFLGWYRQAPGKEREKVAHISIGDQTDYADSAKGRFTISRDESKNMVYLQMNSLKPEDTAVYFCRAFSRIYPYDYWGQGTLVTVSSGGGGSGGGGSGGGGSGGGGSGGGGSGGGGSGGGGSEVQLVESGGGLVQAGGSLRLSCAASGITFSINTMGWYRQAPGKQRELVALISSIGDTYYADSVKGRFTISRDNAKNTVYLQMNSLKPEDTAVYYCKRFRTAAQGTDYWGQGTLVTVSS

SEQ ID NO: 464 - protein, 439 aa, synthetic construct
  REGION 1..439: note = Nanobody sequence
EVQLVESGGGLVQAGGSLRLSCAASGRTFSSYVMGWFRQATGKEREFVATIAWDSGSTYYADSVKGRFTISRDNAKNTVHLQMNSLKPEDTAVYYCAASYNVYYNNYYYPISRDEYDYWGQGTLVTVSSGGGGSGGGGSGGGGSGGGGSGGGGSGGGGSGGGGSEVQLVESGGGSVQAGGSLRLSCAASGDTYGSYWMGWFRQAPGKEREGVAAINRGGGYTVYADSVKGRFTISRDTAKNTVYLQMNSLRPDDTADYYCAASGVLGGLHEDWFNYWGQGTLVTVSSGGGGSGGGGSGGGGSGGGGSGGGGSGGGGSGGGGSEVQLVESGGGLVQPGGSLRLSCVASGDVHKINFLGWYRQAPGKEREKVAHISIGDQTDYADSAKGRFTISRDESKNMVYLQMNSLKPEDTAVYFCRAFSRIYPYDYWGQGTLVTVSS

SEQ ID NO: 465 - protein, 443 aa, synthetic construct
  REGION 1..443: note = Nanobody sequence
EVQLVESGGGSVQAGGSLRLSCAASGYTIGPYCMGWFRQAPGKEREGVAAINMGGGITYYADSVKGRFTISQDNAKNTVYLLMNSLEPEDTAIYYCAADSTIYASYYECGHGLSTGGYGYDSWGQGTLVTVSSGGGGSGGGGSGGGGSGGGGSGGGGSGGGGSGGGGSEVQLVESGGGSVQAGGSLRLSCAASGDTYGSYWMGWFRQAPGKEREGVAAINRGGGYTVYADSVKGRFTISRDTAKNTVYLQMNSLRPDDTADYYCAASGVLGGLHEDWFNYWGQGTLVTVSSGGGGSGGGGSGGGGSGGGGSGGGGSGGGGSGGGGSEVQLVESGGGLVQPGGSLRLSCVASGDVHKINFLGWYRQAPGKEREKVAHISIGDQTDYADSAKGRFTISRDESKNMVYLQMNSLKPEDTAVYFCRAFSRIYPYDYWGQGTLVTVSS

SEQ ID NO: 466 - protein, 449 aa, synthetic construct
  REGION 1..449: note = Nanobody sequence
EVQLVESGGGLVQAGGSLRLSCAASGRTFSSYVMGWFRQATGKEREFVATIAWDSGSTYYADSVKGRFTISRDNAKNTVHLQMNSLKPEDTAVYYCAASYNVYYNNYYYPISRDEYDYWGQGTLVTVSSGGGGSGGGGSGGGGSGGGGSGGGGSGGGGSGGGGSEVQLVESGGGSVQAGGSLRLSCAASGYTIGPYCMGWFRQAPGKEREGVAAINMGGGITYYADSVKGRFTISQDNAKNTVYLLMNSLEPEDTAIYYCAADSTIYASYYECGHGLSTGGYGYDSWGQGTLVTVSSGGGGSGGGGSGGGGSGGGGSGGGGSGGGGSGGGGSEVQLVESGGGLVQPGGSLRLSCVASGDVHKINFLGWYRQAPGKEREKVAHISIGDQTDYADSAKGRFTISRDESKNMVYLQMNSLKPEDTAVYFCRAFSRIYPYDYWGQGTLVTVSS

SEQ ID NO: 467 - protein, 422 aa, synthetic construct
  REGION 1..422: note = Nanobody sequence
DVQLVESGGGLVQPGGSLRLSCTFSGGTFSSYTMGWFRQAPGKEREFVAEVRWGGVTTYSNSLKDRFSISEDSVKNAVYLQMNSLKPEDTAVYYCAAVRQMYMTVVPDYWGQGTLVTVSSGGGGSGGGGSGGGGSGGGGSGGGGSGGGGSGGGGSEVQLVESGGGLVQPGGSLRLSCAASGDVHKINILGWYRQAPAKEREMVAHITIGDATDYADSAKGRFTISRDEAKNMVYLQMNSLKPEDTAVYFCRAYSRIYPYNYWGQGTLVTVSSGGGGSGGGGSGGGGSGGGGSGGGGSGGGGSGGGGSEVQLVESGGGLVQPGNSLRLSCAASGFTFSSFGMSWVRQAPGKGLEWVSSISGSGSDTLYADSVKGRFTISRDNAKTTLYLQMNSLRPEDTAVYYCTIGGSLSRSSQGTLVTVSS

SEQ ID NO: 468 - protein, 272 aa, synthetic construct
  REGION 1..272: note = Nanobody sequence
DVQLVESGGGLVQPGGSLRLSCTFSGGTFSSYTMGWFRQAPGKEREFVAEVRWGGVTTYSNSLKDRFSISEDSVKNAVYLQMNSLKPEDTAVYYCAAVRQMYMTVVPDYWGQGTLVTVSSGGGGSGGGGSGGGGSGGGGSGGGGSGGGGSGGGGSEVQLVESGGGLVQPGGSLRLSCVASGDVHKINFLGWYRQAPGKEREKVAHISIGDQTDYADSAKGRFTISRDESKNMVYLQMNSLKPEDTAVYFCRAFSRIYPYDYWGQGTLVTVSS

SEQ ID NO: 469 - protein, 429 aa, synthetic construct
  REGION 1..429: note = Nanobody sequence
DVQLVESGGGLVQAGDSLRLSCAASGRTFSSYAMGWFRQAPGKEREFVAAISWSDGSTYYADSVKGRFTISRDNAKNTVYLQMNSLKPEDTAVYYCAADLTSTNPGSYIYIWAYDYWGQGTQVTVSSGGGGSGGGGSGGGGSGGGGSGGGGSGGGGSGGGGSEVQLVESGGGLVQPGGSLRLSCAASGDVHKINILGWYRQAPAKEREMVAHITIGDATDYADSAKGRFTISRDEAKNMVYLQMNSLKPEDTAVYFCRAYSRIYPYNYWGQGTLVTVSSGGGGSGGGGSGGGGSGGGGSGGGGSGGGGSGGGGSEVQLVESGGGLVQPGNSLRLSCAASGFTFSSFGMSWVRQAPGKGLEWVSSISGSGSDTLYADSVKGRFTISRDNAKTTLYLQMNSLRPEDTAVYYCTIGGSLSRSSQGTLVTVSS

SEQ ID NO: 470 - protein, 272 aa, synthetic construct
  REGION 1..272: note = Nanobody sequence
DVQLVESGGGLVQPGGSLRLSCTFSGGTFSSYTMGWFRQAPGKEREFVAEVRWGGVTTYSNSLKDRFSISEDSVKNAVYLQMNSLKPEDTAVYYCAAVRQMYMTVVPDYWGQGTLVTVSSGGGGSGGGGSGGGGSGGGGSGGGGSGGGGSGGGGSEVQLVESGGGLVQPGGSLRLSCAASGDVHKINILGWYRQAPAKEREMVAHITIGDATDYADSAKGRFTISRDEAKNMVYLQMNSLKPEDTAVYFCRAYSRIYPYNYWGQGTLVTVSS

SEQ ID NO: 471 - protein, 279 aa, synthetic construct
  REGION 1..279: note = Nanobody sequence
DVQLVESGGGLVQAGDSLRLSCAASGRTFSSYAMGWFRQAPGKEREFVAAISWSDGSTYYADSVKGRFTISRDNAKNTVYLQMNSLKPEDTAVYYCAADLTSTNPGSYIYIWAYDYWGQGTQVTVSSGGGGSGGGGSGGGGSGGGGSGGGGSGGGGSGGGGSEVQLVESGGGLVQPGGSLRLSCAASGDVHKINILGWYRQAPAKEREMVAHITIGDATDYADSAKGRFTISRDEAKNMVYLQMNSLKPEDTAVYFCRAYSRIYPYNYWGQGTLVTVSS

SEQ ID NO: 472 - protein, 10 aa, synthetic construct
  REGION 1..10: note = CDR1
GFTFSSFGMS

SEQ ID NO: 473 - protein, 10 aa, synthetic construct
  REGION 1..10: note = CDR1
GFTFRSFGMS

SEQ ID NO: 474 - protein, 10 aa, synthetic construct
  REGION 1..10: note = CDR2
SISGSGSDTL

SEQ ID NO: 475 - protein, 6 aa, synthetic construct
  REGION 1..6: note = CDR3
GGSLSR

SEQ ID NO: 476 - protein, 110 aa, Homo sapiens
NAGVTQTPKFRILKIGQSMTLQCTQDMNHNYMYWYRQDPGMGLKLIYYSVGAGITDKGEVPNGYNVSRSTTEDFPLRLELAAPSQTSVYFCASTYHGTGYFGEGSWLTVV

SEQ ID NO: 477 - protein, 112 aa, Homo sapiens
DGGITQSPKYLFRKEGQNVTLSCEQNLNHDAMYWYRQDPGQGLRLIYYSQIVNDFQKGDIAEGYSVSREKKESFPLTVTSAQKNPTAFYLCASSSRSSYEQYFGPGTRLTVT

SEQ ID NO: 478 - protein, 114 aa, Homo sapiens
VVSQHPSWVIAKSGTSVKIECRSLDFQATTMFWYRQFPKQSLMLMATSNEGSKATYEQGVEKDKFLINHASLTLSTLTVTSAHPEDSSFYICSARGGSYNSPLHFGNGTRLTVT

SEQ ID NO: 479 - protein, 96 aa, Homo sapiens
PNIQNPDPAVYQLRDSKSSDKSVCLFTDFDSQTNVSQSKDSDVYITDKTVLDMRSMDFKSNSAVAWSNKSDFACANAFNNSIIPEDTFFPSPESSC

SEQ ID NO: 480 - protein, 131 aa, Homo sapiens
EDLNKVFPPEVAVFEPSEAEISHTQKATLVCLATGFFPDHVELSWWVNGKEVHSGVSTDPQPLKEQPALNDSRYCLSSRLRVSATFWQNPRNHFRCQVQFYGLSENDEWTQDRAKPVTQIVSAEAWGRADC

SEQ ID NO: 481 - protein, 5 aa, synthetic construct
  REGION 1..5: note = CDR1
SFGMS

SEQ ID NO: 482 - protein, 17 aa, synthetic construct
  REGION 1..17: note = CDR2
SISGSGSDTLYADSVKG

SEQ ID NO: 483 - protein, 98 aa, synthetic construct
  REGION 1..98: note = Nanobody sequence
QVQLVESGGGLVQPGGSLRLSCAASGFTLDYYAIGWFRQAPGKEREGVSCISSSDGSTYYADSVKGRFTISRDNAKNTVYLQMNSLKPEDTAVYYCAA

SEQ ID NO: 484 - protein, 142 aa, Homo sapiens
PNIQNPDPAVYQLRDSKSSDKSVCLFTDFDSQTNVSQSKDSDVYITDKTVLDMRSMDFKSNSAVAWSNKSDFACANAFNNSIIPEDTFFPSPESSCDVKLVEKSFETDTNLNFQNLSVIGFRILLLKVAGFNLLMTLRLWSS

SEQ ID NO: 485 - protein, 177 aa, Homo sapiens
EDLNKVFPPEVAVFEPSEAEISHTQKATLVCLATGFFPDHVELSWWVNGKEVHSGVSTDPQPLKEQPALNDSRYCLSSRLRVSATFWQNPRNHFRCQVQFYGLSENDEWTQDRAKPVTQIVSAEAWGRADCGFTSVSYQQGVLSATILYEILLGKATLYAVLVSALVLMAMVKRKDF

SEQ ID NO: 486 - protein, 623 aa, synthetic construct
  REGION 1..623: note = Nanobody sequence
EVQLVESGGGLVQAGGSLRLSCAASGRTFSSYVMGWFRQATGKEREFVATIAWDSGSTYYADSVKGRFTISRDNAKNTVHLQMNSLKPEDTAVYYCAASYNVYYNNYYYPISRDEYDYWGQGTLVTVSSGGGGSGGGGSGGGGSGGGGSGGGGSGGGGSGGGGSEVQLVESGGGSVQAGGSLRLSCAASGDTYGSYWMGWFRQAPGKEREGVAAINRGGGYTVYADSVKGRFTISRDTAKNTVYLQMNSLRPDDTADYYCAASGVLGGLHEDWFNYWGQGTLVTVSSGGGGSGGGGSGGGGSGGGGSGGGGSGGGGSGGGGSEVQLVESGGGLVQPGGSLRLSCVASGDVHKINFLGWYRQAPGKEREKVAHISIGDQTDYADSAKGRFTISRDESKNMVYLQMNSLKPEDTAVYFCRAFSRIYPYDYWGQGTLVTVSSGGGGSGGGGSGGGGSGGGGSGGGGSGGGGSGGGGSEVQLVESGGGLVQPGNSLRLSCAASGFTFSSFGMSWVRQAPGKGLEWVSSISGSGSDTLYADSVKGRFTISRDNAKTTLYLQMNSLRPEDTAVYYCTIGGSLSRSSQGTLVTVSSGAADYKDHDGDYKDHDIDYKDDDDKGAAHHHHHH

SEQ ID NO: 487 - protein, 589 aa, synthetic construct
  REGION 1..589: note = Nanobody sequence
EVQLVESGGGLVQAGGSLRLSCAASGRTFSSYVMGWFRQATGKEREFVATIAWDSGSTYYADSVKGRFTISRDNAKNTVHLQMNSLKPEDTAVYYCAASYNVYYNNYYYPISRDEYDYWGQGTLVTVSSGGGGSGGGGSGGGGSGGGGSGGGGSGGGGSGGGGSEVQLVESGGGSVQAGGSLRLSCAASGDTYGSYWMGWFRQAPGKEREGVAAINRGGGYTVYADSVKGRFTISRDTAKNTVYLQMNSLRPDDTADYYCAASGVLGGLHEDWFNYWGQGTLVTVSSGGGGSGGGGSGGGGSGGGGSGGGGSGGGGSGGGGSEVQLVESGGGLVQPGGSLRLSCVASGDVHKINFLGWYRQAPGKEREKVAHISIGDQTDYADSAKGRFTISRDESKNMVYLQMNSLKPEDTAVYFCRAFSRIYPYDYWGQGTLVTVSSGGGGSGGGGSGGGGSGGGGSGGGGSGGGGSGGGGSEVQLVESGGGLVQPGNSLRLSCAASGFTFSSFGMSWVRQAPGKGLEWVSSISGSGSDTLYADSVKGRFTISRDNAKTTLYLQMNSLRPEDTAVYYCTIGGSLSRSSQGTLVTVSS